European Patent Application EP 4 397 764 A1, published July 10, 2024. Title: Gene sequence construct for gene therapy of human immunodeficiency virus infection. Applicant: Kanglin Biotechnology (Hangzhou) Co. Ltd. The sequence listing filed with the application follows.

SEQUENCE LISTING (22 sequences)

SEQ ID NO: 1 - protein, 20 aa, synthetic construct
  REGION 1..20: note = signal peptide
MARPLCTLLLLMATLAGALA

SEQ ID NO: 2 - protein, 254 aa, synthetic construct
  REGION 1..254: note = 10E8v4-5R+100cF scFv
SELTQDPAVSVALKQTVTITCRGDSLRSHYASWYQKKPGQAPVLLFYGKNNRPSGIPDRFSGSASGNRASLTITGAQAEDEADYYCSSRDKSGSRLSVFGGGTKLTVLGGGGSGGGGSGGGGSEVRLRESGGGLVKPGGSLRLSCSASGFDFDNAWMTWVRQPPGKGLEWVGRITGPGEGWSVDYAESVKGRFTISRDNTKNTLYLEMNNVRTEDTGYYFCARTGKYYDFWFGYPPGEEYFQDWGQGTLVIVSS

SEQ ID NO: 3 - protein, 253 aa, synthetic construct
  REGION 1..253: note = Ibalizumab scFv
DIVMTQSPDSLAVSLGERVTMNCKSSQSLLYSTNQKNYLAWYQQKPGQSPKLLIYWASTRESGVPDRFSGSGSGTDFTLTISSVQAEDVAVYYCQQYYSYRTFGGGTKLEIKRTVAGGGGSGGGGSGGGGSQVQLQQSGPEVVKPGASVKMSCKASGYTFTSYVIHWVRQKPGQGLDWIGYINPYNDGTDYDEKFKGKATLTSDTSTSTAYMELSSLRSEDTAVYYCAREKDNYATGAWFAYWGQGTLVTVSS

SEQ ID NO: 4 - protein, 28 aa, synthetic construct
  REGION 1..28: note = HIV membrane fusion-inhibiting peptide P52
WEQKIEELLKKAEEQQKKNEEELKKLEK

SEQ ID NO: 5 - protein, 36 aa, synthetic construct
  REGION 1..36: note = HIV membrane fusion-inhibiting peptide C34
YTSLIHSLIEESQNQQEKNEQELLELDKWASLWNWF

SEQ ID NO: 6 - protein, 34 aa, synthetic construct
  REGION 1..34: note = HIV membrane fusion-inhibiting peptide T20
LLEQENKEQQNQSEEILSHILSTYNNIERDWEMW

SEQ ID NO: 7 - protein, 552 aa, synthetic construct
  REGION 1..552: note = KL-BsHIV01-02
MARPLCTLLLLMATLAGALASELTQDPAVSVALKQTVTITCRGDSLRSHYASWYQKKPGQAPVLLFYGKNNRPSGIPDRFSGSASGNRASLTITGAQAEDEADYYCSSRDKSGSRLSVFGGGTKLTVLGGGGSGGGGSGGGGSEVRLRESGGGLVKPGGSLRLSCSASGFDFDNAWMTWVRQPPGKGLEWVGRITGPGEGWSVDYAESVKGRFTISRDNTKNTLYLEMNNVRTEDTGYYFCARTGKYYDFWFGYPPGEEYFQDWGQGTLVIVSSGGGGSGGGGSGGGGSGGGGSGGGGSDIVMTQSPDSLAVSLGERVTMNCKSSQSLLYSTNQKNYLAWYQQKPGQSPKLLIYWASTRESGVPDRFSGSGSGTDFTLTISSVQAEDVAVYYCQQYYSYRTFGGGTKLEIKRTVAGGGGSGGGGSGGGGSQVQLQQSGPEVVKPGASVKMSCKASGYTFTSYVIHWVRQKPGQGLDWIGYINPYNDGTDYDEKFKGKATLTSDTSTSTAYMELSSLRSEDTAVYYCAREKDNYATGAWFAYWGQGTLVTVSS

SEQ ID NO: 8 - DNA, 1659 bp, synthetic construct
  misc_feature 1..1659: note = KL-BsHIV01-02
  source 1..1659: mol_type = other DNA
atggcgagacccctgtgcacattacttctgttgatggctaccctggcaggcgccctcgccagcgagctgacacaggaccctgccgtgtccgtggccctgaagcagaccgtgacaatcacctgcagaggcgattccctgagatcccactacgcctcctggtaccagaagaagcctggccaggcccccgtgctgctgttttacggcaagaataaccgccccagcggcatccccgatagattttccggcagcgcctccggcaacagagccagcctgacaatcaccggcgcccaggccgaggacgaggctgattactactgcagctccagagataagagcggcagcagactgtccgtgtttggcggcggcaccaagctgaccgtgctcggaggaggaggaagcggaggaggaggctcaggcggcggcggctctgaggtgaggctgagagagtccggcggcggcctggtgaagcccggaggatctctgaggctgtcctgctccgcctccggcttcgattttgacaatgcctggatgacctgggtgagacagccccctggcaagggcctggagtgggtgggaaggatcacaggccccggcgagggctggtccgtggattacgccgagtccgtgaagggcaggttcacaatctccagggataacaccaagaacaccctgtacctggagatgaacaacgtgaggacagaggataccggctactacttttgcgccagaacaggcaagtactacgacttttggttcggctacccccctggcgaggagtacttccaggattggggccagggcaccctggtcattgtgtccagcggcggcggcggcagtggcggcggcggaagcggcggcggcggctctggcggcggcggcagcggcggcggcggctccgacatcgtgatgacccagtctcctgatagcctggccgtgagcctgggcgagagagtgacaatgaactgtaagtctagccagagcctgctgtactccaccaaccagaagaattacctggcctggtatcagcagaagcctggccagtccccaaagctgctgatctattgggcatctacaagggagagcggagtgccagacagattcagcggatccggatctggaaccgacttcaccctgacaatctcctctgtgcaggccgaggacgtggccgtgtactattgccagcagtactatagctacaggacattcggcggcggcaccaagctggagatcaagcgcaccgtggccggaggaggaggatctggcggaggagggtccggcggcggcggctcccaggtgcagctgcagcagagcggaccagaggtggtgaagcctggagcctccgtgaagatgtcttgtaaggccagcggctacaccttcacatcctatgtgatccactgggtgaggcagaagccaggacagggactggactggatcggctacatcaacccttataatgatggcaccgactacgatgagaagtttaagggcaaggccaccctgacatccgataccagcacatccaccgcctatatggagctgagctccctgcggtctgaggacacagccgtgtactattgcgccagagagaaggataactacgcaaccggagcatggttcgcatattggggacagggtaccctggtcaccgtgtctagctag

SEQ ID NO: 9 - protein, 605 aa, synthetic construct
  REGION 1..605: note = KL-BsHIV01-003-02
MARPLCTLLLLMATLAGALASELTQDPAVSVALKQTVTITCRGDSLRSHYASWYQKKPGQAPVLLFYGKNNRPSGIPDRFSGSASGNRASLTITGAQAEDEADYYCSSRDKSGSRLSVFGGGTKLTVLGGGGSGGGGSGGGGSEVRLRESGGGLVKPGGSLRLSCSASGFDFDNAWMTWVRQPPGKGLEWVGRITGPGEGWSVDYAESVKGRFTISRDNTKNTLYLEMNNVRTEDTGYYFCARTGKYYDFWFGYPPGEEYFQDWGQGTLVIVSSGGGGSGGGGSGGGGSGGGGSGGGGSDIVMTQSPDSLAVSLGERVTMNCKSSQSLLYSTNQKNYLAWYQQKPGQSPKLLIYWASTRESGVPDRFSGSGSGTDFTLTISSVQAEDVAVYYCQQYYSYRTFGGGTKLEIKRTVAGGGGSGGGGSGGGGSQVQLQQSGPEVVKPGASVKMSCKASGYTFTSYVIHWVRQKPGQGLDWIGYINPYNDGTDYDEKFKGKATLTSDTSTSTAYMELSSLRSEDTAVYYCAREKDNYATGAWFAYWGQGTLVTVSSGGGGSGGGGSGGGGSGGGGSGGGGSWEQKIEELLKKAEEQQKKNEEELKKLEK

SEQ ID NO: 10 - DNA, 1818 bp, synthetic construct
  misc_feature 1..1818: note = KL-BsHIV01-003-02
  source 1..1818: mol_type = other DNA
atggcgagacccctgtgcacattacttctgttgatggctaccctggcaggcgccctcgccagcgagctgacacaggaccctgccgtgtccgtggccctgaagcagaccgtgacaatcacctgcagaggcgattccctgagatcccactacgcctcctggtaccagaagaagcctggccaggcccccgtgctgctgttttacggcaagaataaccgccccagcggcatccccgatagattttccggcagcgcctccggcaacagagccagcctgacaatcaccggcgcccaggccgaggacgaggctgattactactgcagctccagagataagagcggcagcagactgtccgtgtttggcggcggcaccaagctgaccgtgctcggaggaggaggaagcggaggaggaggctcaggcggcggcggctctgaggtgaggctgagagagtccggcggcggcctggtgaagcccggaggatctctgaggctgtcctgctccgcctccggcttcgattttgacaatgcctggatgacctgggtgagacagccccctggcaagggcctggagtgggtgggaaggatcacaggccccggcgagggctggtccgtggattacgccgagtccgtgaagggcaggttcacaatctccagggataacaccaagaacaccctgtacctggagatgaacaacgtgaggacagaggataccggctactacttttgcgccagaacaggcaagtactacgacttttggttcggctacccccctggcgaggagtacttccaggattggggccagggcaccctggtcattgtgtccagcggcggcggcggcagtggcggcggcggaagcggcggcggcggctctggcggcggcggcagcggcggcggcggctccgacatcgtgatgacccagtctcctgatagcctggccgtgagcctgggcgagagagtgacaatgaactgtaagtctagccagagcctgctgtactccaccaaccagaagaattacctggcctggtatcagcagaagcctggccagtccccaaagctgctgatctattgggcatctacaagggagagcggagtgccagacagattcagcggatccggatctggaaccgacttcaccctgacaatctcctctgtgcaggccgaggacgtggccgtgtactattgccagcagtactatagctacaggacattcggcggcggcaccaagctggagatcaagcgcaccgtggccggaggaggaggatctggcggaggagggtccggcggcggcggctcccaggtgcagctgcagcagagcggaccagaggtggtgaagcctggagcctccgtgaagatgtcttgtaaggccagcggctacaccttcacatcctatgtgatccactgggtgaggcagaagccaggacagggactggactggatcggctacatcaacccttataatgatggcaccgactacgatgagaagtttaagggcaaggccaccctgacatccgataccagcacatccaccgcctatatggagctgagctccctgcggtctgaggacacagccgtgtactattgcgccagagagaaggataactacgcaaccggagcatggttcgcatattggggacagggtaccctggtcaccgtgtctagcggcggaggaggaagcggaggaggcggctctggcggaggaggttccggaggaggcggaagcggcggaggaggctcttgggagcagaagatcgaggagctgctgaagaaggccgaggagcagcagaagaagaatgaggaggagctgaagaagctggagaagtag

SEQ ID NO: 11 - protein, 6709 aa, synthetic construct
  REGION 1..6709: note = pKL-kan-lenti-CBH-WPRE
GGCCGCGTTGCTGGCGTTTTTCCATAGGCTCCGCCCCCCTGACGAGCATCACAAAAATCGACGCTCAAGTCAGAGGTGGCGAAACCCGACAGGACTATAAAGATACCAGGCGTTTCCCCCTGGAAGCTCCCTCGTGCGCTCTCCTGTTCCGACCCTGCCGCTTACCGGATACCTGTCCGCCTTTCTCCCTTCGGGAAGCGTGGCGCTTTCTCATAGCTCACGCTGTAGGTATCTCAGTTCGGTGTAGGTCGTTCGCTCCAAGCTGGGCTGTGTGCACGAACCCCCCGTTCAGCCCGACCGCTGCGCCTTATCCGGTAACTATCGTCTTGAGTCCAACCCGGTAAGACACGACTTATCGCCACTGGCAGCAGCCACTGGTAACAGGATTAGCAGAGCGAGGTATGTAGGCGGTGCTACAGAGTTCTTGAAGTGGTGGCCTAACTACGGCTACACTAGAAGAACAGTATTTGGTATCTGCGCTCTGCTGAAGCCAGTTACCTTCGGAAAAAGAGTTGGTAGCTCTTGATCCGGCAAACAAACCACCGCTGGTAGCGGTGGTTTTTTTGTTTGCAAGCAGCAGATTACGCGCAGAAAAAAAGGATCTCAAGAAGATCCTTTGATCTTTTCTACGGGGTCTGACGCTCAGTGGAACGAAAACTCACGTTAAGGGATTTTGGTCATGAAGCGCTTTTGAAGCTCGGATCCGAACAAACGACCCAACACCCGTGCGTTTTATTCTGTCTTTTTATTGCCGATCCCCTCAGAAGAACTCGTCAAGAAGGCGATAGAAGGCGATGCGCTGCGAATCGGGAGCGGCGATACCGTAAAGCACGAGGAAGCGGTCAGCCCATTCGCCGCCAAGCTCTTCAGCAATATCACGGGTAGCCAACGCTATGTCCTGATAGCGGTCCGCCACACCCAGCCGGCCACAGTCGATGAATCCAGAAAAGCGGCCATTTTCCACCATGATATTCGGCAAGCAGGCATCGCCATGGGTCACGACGAGATCCTCGCCGTCGGGCATGCTCGCCTTGAGCCTGGCGAACAGTTCGGCTGGCGCGAGCCCCTGATGCTCTTCGTCCAGATCATCCTGATCGACAAGACCGGCTTCCATCCGAGTACGTGCTCGCTCGATGCGATGTTTCGCTTGGTGGTCGAATGGGCAGGTAGCCGGATCAAGCGTATGCAGCCGCCGCATTGCATCAGCCATGATGGATACTTTCTCGGCAGGAGCAAGGTGAGATGACAGGAGATCCTGCCCCGGCACTTCGCCCAATAGCAGCCAGTCCCTTCCCGCTTCAGTGACAACGTCGAGCACAGCTGCGCAAGGAACGCCCGTCGTGGCCAGCCACGATAGCCGCGCTGCCTCGTCTTGCAGTTCATTCAGGGCACCGGACAGGTCGGTCTTGACAAAAAGAACCGGGCGCCCCTGCGCTGACAGCCGGAACACGGCGGCATCAGAGCAGCCGATTGTCTGTTGTGCCCAGTCATAGCCGAATAGCCTCTCCACCCAAGCGGCCGGAGAACCTGCGTGCAATCCATCTTGTTCAATCATGCGAAACGATCCTCATCCTGTCTCTTGATCAGAGCTTGATCCCCTGCGCCATCAGATCCTTGGCGGCAAGAAAGCCATCCAGTTTACTTTGCAGGGCTTCCCAACCTTACCAGAGGCCTGCGCCGCGGCCAGCTGGCTAGCAATTCCCGGGTTAACTCTAGAGACATTGATTATTGACTAGTTATTAATAGTAATCAATTACGGGGTCATTAGTTCATAGCCCATATATGGAGTTCCGCGTTACATAACTTACGGTAAATGGCCCGCCTGGCTGACCGCCCAACGACCCCCGCCCATTGACGTCAATAATGACGTATGTTCCCATAGTAACGCCAATAGGGACTTTCCATTGACGTCAATGGGTGGAGTATTTACGGTAAACTGCCCACTTGGCAGTACATCAAGTGTATCATATGCCAAGTACGCCCCCTATTGACGTCAATGACGGTAAATGGCCCGCCTGGCATTATGCCCAGTACATGACCTTATGGGACTTTCCTACTTGGCAGTACATCTACGTATTAGTCATCGCTATTACCATGGTGATGCGGTTTTGGCAGTACATCAATGGGCGTGGATAGCGGTTTGACTCACGGGGATTTCCAAGTCTCCACCCCATTGACGTCAATGGGAGTTTGTTTTGGCACCAAAATCAACGGGACTTTCCAAAATGTCGTAACAACTCCGCCCCATTGACGCAAATGGGCGGTAGGCGTGTACGGTGGGAGGTCTATATAAGCAGAGCTCGTTTAGTGAACCGGGGTCTCTCTGGTTAGACCAGATCTGAGCCTGGGAGCTCTCTGGCTAACTAGGGAACCCACTGCTTAAGCCTCAATAAAGCTTGCCTTGAGTGCTTCAAGTAGTGTGTGCCCGTCTGTTGTGTGACTCTGGTAACTAGAGATCCCTCAGACCCTTTTAGTCAGTGTGGAAAATCTCTAGCAGTGGCGCCCGAACAGGGACTTGAAAGCGAAAGGGAAACCAGAGGAGCTCTCTCGACGCAGGACTCGGCTTGCTGAAGCGCGCACGGCAAGAGGCGAGGGGCGGCGACTGGTGAGTACGCCAAAAATTTTGACTAGCGGAGGCTAGAAGGAGAGAGATGGGTGCGAGAGCGTCAGTATTAAGCGGGGGAGAATTAGATCGCGATGGGAAAAAATTCGGTTAAGGCCAGGGGGAAAGAAAAAATATAAATTAAAACATATAGTATGGGCAAGCAGGGAGCTAGAACGATTCGCAGTTAATCCTGGCCTGTTAGAAACATCAGAAGGCTGTAGACAAATACTGGGACAGCTACAACCATCCCTTCAGACAGGATCAGAAGAACTTAGATCATTATATAATACAGTAGCAACCCTCTATTGTGTGCATCAAAGGATAGAGATAAAAGACACCAAGGAAGCTTTAGACAAGATAGAGGAAGAGCAAAACAAAAGTAAGACCACCGCACAGCAAGCGGCCGCTGATCTTCAGACCTGGAGGAGGAGATATGAGGGACAATTGGAGAAGTGAATTATATAAATATAAAGTAGTAAAAATTGAACCATTAGGAGTAGCACCCACCAAGGCAAAGAGAAGAGTGGTGCAGAGAGAAAAAAGAGCAGTGGGAATAGGAGCTTTGTTCCTTGGGTTCTTGGGAGCAGCAGGAAGCACTATGGGCGCAGCGTCAATGACGCTGACGGTACAGGCCAGACAATTATTGTCTGGTATAGTGCAGCAGCAGAACAATTTGCTGAGGGCTATTGAGGCGCAACAGCATCTGTTGCAACTCACAGTCTGGGGCATCAAGCAGCTCCAGGCAAGAATCCTGGCTGTGGAAAGATACCTAAAGGATCAACAGCTCCTGGGGATTTGGGGTTGCTCTGGAAAACTCATTTGCACCACTGCTGTGCCTTGGAATGCTAGTTGGAGTAATAAATCTCTGGAACAGATTTGGAATCACACGACCTGGATGGAGTGGGACAGAGAAATTAACAATTACACAAGCTTAATACACTCCTTAATTGAAGAATCGCAAAACCAGCAAGAAAAGAATGAACAAGAATTATTGGAATTAGATAAATGGGCAAGTTTGTGGAATTGGTTTAACATAACAAATTGGCTGTGGTATATAAAATTATTCATAATGATAGTAGGAGGCTTGGTAGGTTTAAGAATAGTTTTTGCTGTACTTTCTATAGTGAATAGAGTTAGGCAGGGATATTCACCATTATCGTTTCAGACCCACCTCCCAACCCCGAGGGGACCCGACAGGCCCGAAGGAATAGAAGAAGAAGGTGGAGAGAGAGACAGAGACAGATCCATTCGATTAGTGAACGGATCTCGACGGTATCGGTTAACTTTTAAAAGAAAAGGGGGGATTGGGGGGTACAGTGCAGGGGAAAGAATAGTAGACATAATAGCAACAGACATACAAACTAAAGAATTACAAAAACAAATTACAAAAATTCAAAATTTTATCGATCACGAGACTAGCCTCGAGGCATGCCTGCAGGAATTCGTTACATAACTTACGGTAAATGGCCCGCCTGGCTGACCGCCCAACGACCCCCGCCCATTGACGTCAATAGTAACGCCAATAGGGACTTTCCATTGACGTCAATGGGTGGAGTATTTACGGTAAACTGCCCACTTGGCAGTACATCAAGTGTATCATATGCCAAGTACGCCCCCTATTGACGTCAATGACGGTAAATGGCCCGCCTGGCATTGTGCCCAGTACATGACCTTATGGGACTTTCCTACTTGGCAGTACATCTACGTATTAGTCATCGCTATTACCATGGTCGAGGTGAGCCCCACGTTCTGCTTCACTCTCCCCATCTCCCCCCCCTCCCCACCCCCAATTTTGTATTTATTTATTTTTTAATTATTTTGTGCAGCGATGGGGGCGGGGGGGGGGGGGGGGCGCGCGCCAGGCGGGGCGGGGCGGGGCGAGGGGCGGGGCGGGGCGAGGCGGAGAGGTGCGGCGGCAGCCAATCAGAGCGGCGCGCTCCGAAAGTTTCCTTTTATGGCGAGGCGGCGGCGGCGGCGGCCCTATAAAAAGCGAAGCGCGCGGCGGGCGGGAGTCGCTGCGACGCTGCCTTCGCCCCGTGCCCCGCTCCGCCGCCGCCTCGCGCCGCCCGCCCCGGCTCTGACTGACCGCGTTACTCCCACAGGTGAGCGGGCGGGACGGCCCTTCTCCTCCGGGCTGTAATTAGCTGAGCAAGAGGTAAGGGTTTAAGGGATGGTTGGTTGGTGGGGTATTAATGTTTAATTACCTGGAGCACCTGCCTGAAATCACTTTTTTTCAGGTTGGACCGGTACGCGTGCCTCGGATCCTCCAGTGTGGTGTGCAGATATCCAGCACAGTCCCGGGCCGAGTCTAGACGTTTAAACCCGCTGATCAGGTCGACAATCAACCTCTGGATTACAAAATTTGTGAAAGATTGACTGGTATTCTTAACTATGTTGCTCCTTTTACGCTATGTGGATACGCTGCTTTAATGCCTTTGTATCATGCTATTGCTTCCCGTATGGCTTTCATTTTCTCCTCCTTGTATAAATCCTGGTTGCTGTCTCTTTATGAGGAGTTGTGGCCCGTTGTCAGGCAACGTGGCGTGGTGTGCACTGTGTTTGCTGACGCAACCCCCACTGGTTGGGGCATTGCCACCACCTGTCAGCTCCTTTCCGGGACTTTCGCTTTCCCCCTCCCTATTGCCACGGCGGAACTCATCGCCGCCTGCCTTGCCCGCTGCTGGACAGGGGCTCGGCTGTTGGGCACTGACAATTCCGTGGTGTTGTCGGGGAAGCTGACGTCCTTTCCATGGCTGCTCGCCTGTGTTGCCACCTGGATTCTGCGCGGGACGTCCTTCTGCTACGTCCCTTCGGCCCTCAATCCAGCGGACCTTCCTTCCCGCGGCCTGCTGCCGGCTCTGCGGCCTCTTCCGCGTCTTCGCCTTCGCCCTCAGACGAGTCGGATCTCCCTTTGGGCCGCCTCCCCGCGGTACCTTTAAGACCAATGACTTACAAGGCAGCTGTAGATCTTAGCCACTTTTTAAAAGAAAAGGGGGGACTGGAAGGGCTAATTCACTCCCAACGAAGACAAGATCTGCTTTTTGCTTGTACTGGGTCTCTCTGGTTAGACCAGATCTGAGCCTGGGAGCTCTCTGGCTAACTAGGGAACCCACTGCTTAAGCCTCAATAAAGCTTGCCTTGAGTGCTTCAAGTAGTGTGTGCCCGTCTGTTGTGTGACTCTGGTAACTAGAGATCCCTCAGACCCTTTTAGTCAGTGTGGAAAATCTCTAGCAGTAGTAGTTCATGTCATCTTATTATTCAGTATTTATAACTTGCAAAGAAATGAATATCAGAGAGTGAGAGGAACTTGTTTATTGCAGCTTATAATGGTTACAAATAAAGCAATAGCATCACAAATTTCACAAATAAAGCATTTTTTTCACTGCATTCTAGTTGTGGTTTGTCCAAACTCATCAATGTATCTTATCATGTCTGGCTCTAGCTATCCCGCCCCTAACTCCGCCCATCCCGCCCCTAACTCCGCCCAGTTCCGCCCATTCTCCGCCCCATGGCTGACTAATTTTTTTTATTTATGCAGAGGCCGAGGCCGCCTCGGCCTCTGAGCTATTCCAGAAGTAGTGAGGAGGCTTTTTTGGAGGCCGCTAGCGTCGACCATTACTTATTGTTTTAGCTGTCCTCATGAATGTCTTTTCACTACCCATTTGCTTATCCTGCATCTCTCAGCCTTGACTCCACTCAGTTCTCTTGCTTAGAGATACCACCTTTCCCCTGAAGTGTTCCTTCCATGTTTTACGGCGAGATGGTTTCTCCTCGCCTGGCCACTCAGCCTTAGTTGTCTCTGTTGTCTTATAGAGGTCTACTTGAAGAAGGAAAAACAGGGGGCATGGTTTGACTGTCCTGTGAGCCCTTCTTCCCTGCCTCCCCCACTCACAGTGACCCGGAATCCCTCGACATGGCAGTCTAGCACTAGTGCGGCCGCAGATCTGCTTCCTCGCTCACTGACTCGCTGCGCTCGGTCGTTCGGCTGCGGCGAGCGGTATCAGCTCACTCAAAGGCGGTAATACGGTTATCCACAGAATCAGGGGATAACGCAGGAAAGAACATGTGAGCAAAAGGCCAGCAAAAGGCCAGGAACCGTAAAAA

SEQ ID NO: 12 - DNA, 8305 bp, synthetic construct
  misc_feature 1..8305: note = pKL-Kan-lenti-CBH-KL-BsHIV01-02
  source 1..8305: mol_type = other DNA
ggccgcgttgctggcgtttttccataggctccgcccccctgacgagcatcacaaaaatcgacgctcaagtcagaggtggcgaaacccgacaggactataaagataccaggcgtttccccctggaagctccctcgtgcgctctcctgttccgaccctgccgcttaccggatacctgtccgcctttctcccttcgggaagcgtggcgctttctcatagctcacgctgtaggtatctcagttcggtgtaggtcgttcgctccaagctgggctgtgtgcacgaaccccccgttcagcccgaccgctgcgccttatccggtaactatcgtcttgagtccaacccggtaagacacgacttatcgccactggcagcagccactggtaacaggattagcagagcgaggtatgtaggcggtgctacagagttcttgaagtggtggcctaactacggctacactagaagaacagtatttggtatctgcgctctgctgaagccagttaccttcggaaaaagagttggtagctcttgatccggcaaacaaaccaccgctggtagcggtggtttttttgtttgcaagcagcagattacgcgcagaaaaaaaggatctcaagaagatcctttgatcttttctacggggtctgacgctcagtggaacgaaaactcacgttaagggattttggtcatgaagcgcttttgaagctcggatccgaacaaacgacccaacacccgtgcgttttattctgtctttttattgccgatcccctcagaagaactcgtcaagaaggcgatagaaggcgatgcgctgcgaatcgggagcggcgataccgtaaagcacgaggaagcggtcagcccattcgccgccaagctcttcagcaatatcacgggtagccaacgctatgtcctgatagcggtccgccacacccagccggccacagtcgatgaatccagaaaagcggccattttccaccatgatattcggcaagcaggcatcgccatgggtcacgacgagatcctcgccgtcgggcatgctcgccttgagcctggcgaacagttcggctggcgcgagcccctgatgctcttcgtccagatcatcctgatcgacaagaccggcttccatccgagtacgtgctcgctcgatgcgatgtttcgcttggtggtcgaatgggcaggtagccggatcaagcgtatgcagccgccgcattgcatcagccatgatggatactttctcggcaggagcaaggtgagatgacaggagatcctgccccggcacttcgcccaatagcagccagtcccttcccgcttcagtgacaacgtcgagcacagctgcgcaaggaacgcccgtcgtggccagccacgatagccgcgctgcctcgtcttgcagttcattcagggcaccggacaggtcggtcttgacaaaaagaaccgggcgcccctgcgctgacagccggaacacggcggcatcagagcagccgattgtctgttgtgcccagtcatagccgaatagcctctccacccaagcggccggagaacctgcgtgcaatccatcttgttcaatcatgcgaaacgatcctcatcctgtctcttgatcagagcttgatcccctgcgccatcagatccttggcggcaagaaagccatccagtttactttgcagggcttcccaaccttaccagaggcctgcgccgcggccagctggctagcaattcccgggttaactctagagacattgattattgactagttattaatagtaatcaattacggggtcattagttcatagcccatatatggagttccgcgttacataacttacggtaaatggcccgcctggctgaccgcccaacgacccccgcccattgacgtcaataatgacgtatgttcccatagtaacgccaatagggactttccattgacgtcaatgggtggagtatttacggtaaactgcccacttggcagtacatcaagtgtatcatatgccaagtacgccccctattgacgtcaatgacggtaaatggcccgcctggcattatgcccagtacatgaccttatgggactttcctacttggcagtacatctacgtattagtcatcgctattaccatggtgatgcggttttggcagtacatcaatgggcgtggatagcggtttgactcacggggatttccaagtctccaccccattgacgtcaatgggagtttgttttggcaccaaaatcaacgggactttccaaaatgtcgtaacaactccgccccattgacgcaaatgggcggtaggcgtgtacggtgggaggtctatataagcagagctcgtttagtgaaccggggtctctctggttagaccagatctgagcctgggagctctctggctaactagggaacccactgcttaagcctcaataaagcttgccttgagtgcttcaagtagtgtgtgcccgtctgttgtgtgactctggtaactagagatccctcagacccttttagtcagtgtggaaaatctctagcagtggcgcccgaacagggacttgaaagcgaaagggaaaccagaggagctctctcgacgcaggactcggcttgctgaagcgcgcacggcaagaggcgaggggcggcgactggtgagtacgccaaaaattttgactagcggaggctagaaggagagagatgggtgcgagagcgtcagtattaagcgggggagaattagatcgcgatgggaaaaaattcggttaaggccagggggaaagaaaaaatataaattaaaacatatagtatgggcaagcagggagctagaacgattcgcagttaatcctggcctgttagaaacatcagaaggctgtagacaaatactgggacagctacaaccatcccttcagacaggatcagaagaacttagatcattatataatacagtagcaaccctctattgtgtgcatcaaaggatagagataaaagacaccaaggaagctttagacaagatagaggaagagcaaaacaaaagtaagaccaccgcacagcaagcggccgctgatcttcagacctggaggaggagatatgagggacaattggagaagtgaattatataaatataaagtagtaaaaattgaaccattaggagtagcacccaccaaggcaaagagaagagtggtgcagagagaaaaaagagcagtgggaataggagctttgttccttgggttcttgggagcagcaggaagcactatgggcgcagcgtcaatgacgctgacggtacaggccagacaattattgtctggtatagtgcagcagcagaacaatttgctgagggctattgaggcgcaacagcatctgttgcaactcacagtctggggcatcaagcagctccaggcaagaatcctggctgtggaaagatacctaaaggatcaacagctcctggggatttggggttgctctggaaaactcatttgcaccactgctgtgccttggaatgctagttggagtaataaatctctggaacagatttggaatcacacgacctggatggagtgggacagagaaattaacaattacacaagcttaatacactccttaattgaagaatcgcaaaaccagcaagaaaagaatgaacaagaattattggaattagataaatgggcaagtttgtggaattggtttaacataacaaattggctgtggtatataaaattattcataatgatagtaggaggcttggtaggtttaagaatagtttttgctgtactttctatagtgaatagagttaggcagggatattcaccattatcgtttcagacccacctcccaaccccgaggggacccgacaggcccgaaggaatagaagaagaaggtggagagagagacagagacagatccattcgattagtgaacggatctcgacggtatcggttaacttttaaaagaaaaggggggattggggggtacagtgcaggggaaagaatagtagacataatagcaacagacatacaaactaaagaattacaaaaacaaattacaaaaattcaaaattttatcgatcacgagactagcctcgaggcatgcctgcaggaattccgttacataacttacggtaaatggcccgcctggctgaccgcccaacgacccccgcccattgacgtcaataatgacgtatgttcccatagtaacgccaatagggactttccattgacgtcaatgggtggagtatttacggtaaactgcccacttggcagtacatcaagtgtatcatatgccaagtacgccccctattgacgtcaatgacggtaaatggcccgcctggcattatgcccagtacatgaccttatgggactttcctacttggcagtacatctacgtattagtcatcgctattaccatggtcgaggtgagccccacgttctgcttcactctccccatctcccccccctccccacccccaattttgtatttatttattttttaattattttgtgcagcgatgggggcggggggggggggggggcgcgcgccaggcggggcggggcggggcgaggggcggggcggggcgaggcggagaggtgcggcggcagccaatcagagcggcgcgctccgaaagtttccttttatggcgaggcggcggcggcggcggccctataaaaagcgaagcgcgcggcgggcgggagtcgctgcgacgctgccttcgccccgtgccccgctccgccgccgcctcgcgccgcccgccccggctctgactgaccgcgttactcccacaggtgagcgggcgggacggcccttctcctccgggctgtaattagctgagcaagaggtaagggtttaagggatggttggttggtggggtattaatgtttaattacctggagcacctgcctgaaatcactttttttcaggtaccggtgccaccatggcgagacccctgtgcacattacttctgttgatggctaccctggcaggcgccctcgccagcgagctgacacaggaccctgccgtgtccgtggccctgaagcagaccgtgacaatcacctgcagaggcgattccctgagatcccactacgcctcctggtaccagaagaagcctggccaggcccccgtgctgctgttttacggcaagaataaccgccccagcggcatccccgatagattttccggcagcgcctccggcaacagagccagcctgacaatcaccggcgcccaggccgaggacgaggctgattactactgcagctccagagataagagcggcagcagactgtccgtgtttggcggcggcaccaagctgaccgtgctcggaggaggaggaagcggaggaggaggctcaggcggcggcggctctgaggtgaggctgagagagtccggcggcggcctggtgaagcccggaggatctctgaggctgtcctgctccgcctccggcttcgattttgacaatgcctggatgacctgggtgagacagccccctggcaagggcctggagtgggtgggaaggatcacaggccccggcgagggctggtccgtggattacgccgagtccgtgaagggcaggttcacaatctccagggataacaccaagaacaccctgtacctggagatgaacaacgtgaggacagaggataccggctactacttttgcgccagaacaggcaagtactacgacttttggttcggctacccccctggcgaggagtacttccaggattggggccagggcaccctggtcattgtgtccagcggcggcggcggcagtggcggcggcggaagcggcggcggcggctctggcggcggcggcagcggcggcggcggctccgacatcgtgatgacccagtctcctgatagcctggccgtgagcctgggcgagagagtgacaatgaactgtaagtctagccagagcctgctgtactccaccaaccagaagaattacctggcctggtatcagcagaagcctggccagtccccaaagctgctgatctattgggcatctacaagggagagcggagtgccagacagattcagcggatccggatctggaaccgacttcaccctgacaatctcctctgtgcaggccgaggacgtggccgtgtactattgccagcagtactatagctacaggacattcggcggcggcaccaagctggagatcaagcgcaccgtggccggaggaggaggatctggcggaggagggtccggcggcggcggctcccaggtgcagctgcagcagagcggaccagaggtggtgaagcctggagcctccgtgaagatgtcttgtaaggccagcggctacaccttcacatcctatgtgatccactgggtgaggcagaagccaggacagggactggactggatcggctacatcaacccttataatgatggcaccgactacgatgagaagtttaagggcaaggccaccctgacatccgataccagcacatccaccgcctatatggagctgagctccctgcggtctgaggacacagccgtgtactattgcgccagagagaaggataactacgcaaccggagcatggttcgcatattggggacagggtaccctggtcaccgtgtctagctaggtcgacaatcaacctctggattacaaaatttgtgaaagattgactggtattcttaactatgttgctccttttacgctatgtggatacgctgctttaatgcctttgtatcatgctattgcttcccgtatggctttcattttctcctccttgtataaatcctggttgctgtctctttatgaggagttgtggcccgttgtcaggcaacgtggcgtggtgtgcactgtgtttgctgacgcaacccccactggttggggcattgccaccacctgtcagctcctttccgggactttcgctttccccctccctattgccacggcggaactcatcgccgcctgccttgcccgctgctggacaggggctcggctgttgggcactgacaattccgtggtgttgtcggggaagctgacgtcctttccatggctgctcgcctgtgttgccacctggattctgcgcgggacgtccttctgctacgtcccttcggccctcaatccagcggaccttccttcccgcggcctgctgccggctctgcggcctcttccgcgtcttcgccttcgccctcagacgagtcggatctccctttgggccgcctccccgcggtacctttaagaccaatgacttacaaggcagctgtagatcttagccactttttaaaagaaaaggggggactggaagggctaattcactcccaacgaagacaagatctgctttttgcttgtactgggtctctctggttagaccagatctgagcctgggagctctctggctaactagggaacccactgcttaagcctcaataaagcttgccttgagtgcttcaagtagtgtgtgcccgtctgttgtgtgactctggtaactagagatccctcagacccttttagtcagtgtggaaaatctctagcagtagtagttcatgtcatcttattattcagtatttataacttgcaaagaaatgaatatcagagagtgagaggaacttgtttattgcagcttataatggttacaaataaagcaatagcatcacaaatttcacaaataaagcatttttttcactgcattctagttgtggtttgtccaaactcatcaatgtatcttatcatgtctggctctagctatcccgcccctaactccgcccatcccgcccctaactccgcccagttccgcccattctccgccccatggctgactaattttttttatttatgcagaggccgaggccgcctcggcctctgagctattccagaagtagtgaggaggcttttttggaggccgctagcgtcgaccattacttattgttttagctgtcctcatgaatgtcttttcactacccatttgcttatcctgcatctctcagccttgactccactcagttctcttgcttagagataccacctttcccctgaagtgttccttccatgttttacggcgagatggtttctcctcgcctggccactcagccttagttgtctctgttgtcttatagaggtctacttgaagaaggaaaaacagggggcatggtttgactgtcctgtgagcccttcttccctgcctcccccactcacagtgacccggaatccctcgacatggcagtctagcactagtgcggccgcagatctgcttcctcgctcactgactcgctgcgctcggtcgttcggctgcggcgagcggtatcagctcactcaaaggcggtaatacggttatccacagaatcaggggataacgcaggaaagaacatgtgagcaaaaggccagcaaaaggccaggaaccgtaaaaa

SEQ ID NO: 13 - DNA, 8517 bp, synthetic construct
  misc_feature 1..8517: note = pKL-Kan-lenti-CBH-KL-BsHIV01-003-02
  source 1..8517: mol_type = other DNA
ggccgcgttgctggcgtttttccataggctccgcccccctgacgagcatcacaaaaatcgacgctcaagtcagaggtggcgaaacccgacaggactataaagataccaggcgtttccccctggaagctccctcgtgcgctctcctgttccgaccctgccgcttaccggatacctgtccgcctttctcccttcgggaagcgtggcgctttctcatagctcacgctgtaggtatctcagttcggtgtaggtcgttcgctccaagctgggctgtgtgcacgaaccccccgttcagcccgaccgctgcgccttatccggtaactatcgtcttgagtccaacccggtaagacacgacttatcgccactggcagcagccactggtaacaggattagcagagcgaggtatgtaggcggtgctacagagttcttgaagtggtggcctaactacggctacactagaagaacagtatttggtatctgcgctctgctgaagccagttaccttcggaaaaagagttggtagctcttgatccggcaaacaaaccaccgctggtagcggtggtttttttgtttgcaagcagcagattacgcgcagaaaaaaaggatctcaagaagatcctttgatcttttctacggggtctgacgctcagtggaacgaaaactcacgttaagggattttggtcatgaagcgcttttgaagctcggatccgaacaaacgacccaacacccgtgcgttttattctgtctttttattgccgatcccctcagaagaactcgtcaagaaggcgatagaaggcgatgcgctgcgaatcgggagcggcgataccgtaaagcacgaggaagcggtcagcccattcgccgccaagctcttcagcaatatcacgggtagccaacgctatgtcctgatagcggtccgccacacccagccggccacagtcgatgaatccagaaaagcggccattttccaccatgatattcggcaagcaggcatcgccatgggtcacgacgagatcctcgccgtcgggcatgctcgccttgagcctggcgaacagttcggctggcgcgagcccctgatgctcttcgtccagatcatcctgatcgacaagaccggcttccatccgagtacgtgctcgctcgatgcgatgtttcgcttggtggtcgaatgggcaggtagccggatcaagcgtatgcagccgccgcattgcatcagccatgatggatactttctcggcaggagcaaggtgagatgacaggagatcctgccccggcacttcgcccaatagcagccagtcccttcccgcttcagtgacaacgtcgagcacagctgcgcaaggaacgcccgtcgtggccagccacgatagccgcgctgcctcgtcttgcagttcattcagggcaccggacaggtcggtcttgacaaaaagaaccgggcgcccctgcgctgacagccggaacacggcggcatcagagcagccgattgtctgttgtgcccagtcatagccgaatagcctctccacccaagcggccggagaacctgcgtgcaatccatcttgttcaatcatgcgaaacgatcctcatcctgtctcttgatcagagcttgatcccctgcgccatcagatccttggcggcaagaaagccatccagtttactttgcagggcttcccaaccttaccagaggcctgcgccgcggccagctggctagcaattcccgggttaactctagagacattgattattgactagttattaatagtaatcaattacggggtcattagttcatagcccatatatggagttccgcgttacataacttacggtaaatggcccgcctggctgaccgcccaacgacccccgcccattgacgtcaataatgacgtatgttcccatagtaacgccaatagggactttccattgacgtcaatgggtggagtatttacggtaaactgcccacttggcagtacatcaagtgtatcatatgccaagtacgccccctattgacgtcaatgacggtaaatggcccgcctggcattatgcccagtacatgaccttatgggactttcctacttggcagtacatctacgtattagtcatcgctattaccatggtgatgcggttttggcagtacatcaatgggcgtggatagcggtttgactcacggggatttccaagtctccaccccattgacgtcaatgggagtttgttttggcaccaaaatcaacgggactttccaaaatgtcgtaacaactccgccccattgacgcaaatgggcggtaggcgtgtacggtgggaggtctatataagcagagctcgtttagtgaaccggggtctctctggttagaccagatctgagcctgggagctctctggctaactagggaacccactgcttaagcctcaataaagcttgccttgagtgcttcaagtagtgtgtgcccgtctgttgtgtgactctggtaactagagatccctcagacccttttagtcagtgtggaaaatctctagcagtggcgcccgaacagggacttgaaagcgaaagggaaaccagaggagctctctcgacgcaggactcggcttgctgaagcgcgcacggcaagaggcgaggggcggcgactggtgagtacgccaaaaattttgactagcggaggctagaaggagagagatgggtgcgagagcgtcagtattaagcgggggagaattagatcgcgatgggaaaaaattcggttaaggccagggggaaagaaaaaatataaattaaaacatatagtatgggcaagcagggagctagaacgattcgcagttaatcctggcctgttagaaacatcagaaggctgtagacaaatactgggacagctacaaccatcccttcagacaggatcagaagaacttagatcattatataatacagtagcaaccctctattgtgtgcatcaaaggatagagataaaagacaccaaggaagctttagacaagatagaggaagagcaaaacaaaagtaagaccaccgcacagcaagcggccgctgatcttcagacctggaggaggagatatgagggacaattggagaagtgaattatataaatataaagtagtaaaaattgaaccattaggagtagcacccaccaaggcaaagagaagagtggtgcagagagaaaaaagagcagtgggaataggagctttgttccttgggttcttgggagcagcaggaagcactatgggcgcagcgtcaatgacgctgacggtacaggccagacaattattgtctggtatagtgcagcagcagaacaatttgctgagggctattgaggcgcaacagcatctgttgcaactcacagtctggggcatcaagcagctccaggcaagaatcctggctgtggaaagatacctaaaggatcaacagctcctggggatttggggttgctctggaaaactcatttgcaccactgctgtgccttggaatgctagttggagtaataaatctctggaacagatttggaatcacacgacctggatggagtgggacagagaaattaacaattacacaagcttaatacactccttaattgaagaatcgcaaaaccagcaagaaaagaatgaacaagaattattggaattagataaatgggcaagtttgtggaattggtttaacataacaaattggctgtggtatataaaattattcataatgatagtaggaggcttggtaggtttaagaatagtttttgctgtactttctatagtgaatagagttaggcagggatattcaccattatcgtttcagacccacctcccaaccccgaggggacccgacaggcccgaaggaatagaagaagaaggtggagagagagacagagacagatccattcgattagtgaacggatctcgacggtatcggttaacttttaaaagaaaaggggggattggggggtacagtgcaggggaaagaatagtagacataatagcaacagacatacaaactaaagaattacaaaaacaaattacaaaaattcaaaattttatcgatcacgagactagcctcgaggcatgcctgcaggaattccgttacataacttacggtaaatggcccgcctggctgaccgcccaacgacccccgcccattgacgtcaataatgacgtatgttcccatagtaacgccaatagggactttccattgacgtcaatgggtggagtatttacggtaaactgcccacttggcagtacatcaagtgtatcatatgccaagtacgccccctattgacgtcaatgacggtaaatggcccgcctggcattatgcccagtacatgaccttatgggactttcctacttggcagtacatctacgtattagtcatcgctattaccatggtcgaggtgagccccacgttctgcttcactctccccatctcccccccctccccacccccaattttgtatttatttattttttaattattttgtgcagcgatgggggcggggggggggggggggcgcgcgccaggcggggcggggcggggcgaggggcggggcggggcgaggcggagaggtgcggcggcagccaatcagagcggcgcgctccgaaagtttccttttatggcgaggcggcggcggcggcggccctataaaaagcgaagcgcgcggcgggcgggagtcgctgcgacgctgccttcgccccgtgccccgctccgccgccgcctcgcgccgcccgccccggctctgactgaccgcgttactcccacaggtgagcgggcgggacggcccttctcctccgggctgtaattagctgagcaagaggtaagggtttaagggatggttggttggtggggtattaatgtttaattacctggagcacctgcctgaaatcactttttttcaggtaccggtcgccaccatggcgagacccctgtgcacattacttctgttgatggctaccctggcaggcgccctcgccagcgagctgacacaggaccctgccgtgtccgtggccctgaagcagaccgtgacaatcacctgcagaggcgattccctgagatcccactacgcctcctggtaccagaagaagcctggccaggcccccgtgctgctgttttacggcaagaataaccgccccagcggcatccccgatagattttccggcagcgcctccggcaacagagccagcctgacaatcaccggcgcccaggccgaggacgaggctgattactactgcagctccagagataagagcggcagcagactgtccgtgtttggcggcggcaccaagctgaccgtgctcggaggaggaggaagcggaggaggaggctcaggcggcggcggctctgaggtgaggctgagagagtccggcggcggcctggtgaagcccggaggatctctgaggctgtcctgctccgcctccggcttcgattttgacaatgcctggatgacctgggtgagacagccccctggcaagggcctggagtgggtgggaaggatcacaggccccggcgagggctggtccgtggattacgccgagtccgtgaagggcaggttcacaatctccagggataacaccaagaacaccctgtacctggagatgaacaacgtgaggacagaggataccggctactacttttgcgccagaacaggcaagtactacgacttttggttcggctacccccctggcgaggagtacttccaggattggggccagggcaccctggtcattgtgtccagcggcggcggcggcagtggcggcggcggaagcggcggcggcggctctggcggcggcggcagcggcggcggcggctccgacatcgtgatgacccagtctcctgatagcctggccgtgagcctgggcgagagagtgacaatgaactgtaagtctagccagagcctgctgtactccaccaaccagaagaattacctggcctggtatcagcagaagcctggccagtccccaaagctgctgatctattgggcatctacaagggagagcggagtgccagacagattcagcggatccggatctggaaccgacttcaccctgacaatctcctctgtgcaggccgaggacgtggccgtgtactattgccagcagtactatagctacaggacattcggcggcggcaccaagctggagatcaagcgcaccgtggccggaggaggaggatctggcggaggagggtccggcggcggcggctcccaggtgcagctgcagcagagcggaccagaggtggtgaagcctggagcctccgtgaagatgtcttgtaaggccagcggctacaccttcacatcctatgtgatccactgggtgaggcagaagccaggacagggactggactggatcggctacatcaacccttataatgatggcaccgactacgatgagaagtttaagggcaaggccaccctgacatccgataccagcacatccaccgcctatatggagctgagctccctgcggtctgaggacacagccgtgtactattgcgccagagagaaggataactacgcaaccggagcatggttcgcatattggggacagggtaccctggtcaccgtgtctagcggcggaggaggaagcggaggaggcggctctggcggaggaggttccggaggaggcggaagcggcggaggaggctcttgggagcagaagatcgaggagctgctgaagaaggccgaggagcagcagaagaagaatgaggaggagctgaagaagctggagaagtaggatatccagcacagtcccgggccgagtctagacgtttaaacccgctgatcaggtcgacaatcaacctctggattacaaaatttgtgaaagattgactggtattcttaactatgttgctccttttacgctatgtggatacgctgctttaatgcctttgtatcatgctattgcttcccgtatggctttcattttctcctccttgtataaatcctggttgctgtctctttatgaggagttgtggcccgttgtcaggcaacgtggcgtggtgtgcactgtgtttgctgacgcaacccccactggttggggcattgccaccacctgtcagctcctttccgggactttcgctttccccctccctattgccacggcggaactcatcgccgcctgccttgcccgctgctggacaggggctcggctgttgggcactgacaattccgtggtgttgtcggggaagctgacgtcctttccatggctgctcgcctgtgttgccacctggattctgcgcgggacgtccttctgctacgtcccttcggccctcaatccagcggaccttccttcccgcggcctgctgccggctctgcggcctcttccgcgtcttcgccttcgccctcagacgagtcggatctccctttgggccgcctccccgcggtacctttaagaccaatgacttacaaggcagctgtagatcttagccactttttaaaagaaaaggggggactggaagggctaattcactcccaacgaagacaagatctgctttttgcttgtactgggtctctctggttagaccagatctgagcctgggagctctctggctaactagggaacccactgcttaagcctcaataaagcttgccttgagtgcttcaagtagtgtgtgcccgtctgttgtgtgactctggtaactagagatccctcagacccttttagtcagtgtggaaaatctctagcagtagtagttcatgtcatcttattattcagtatttataacttgcaaagaaatgaatatcagagagtgagaggaacttgtttattgcagcttataatggttacaaataaagcaatagcatcacaaatttcacaaataaagcatttttttcactgcattctagttgtggtttgtccaaactcatcaatgtatcttatcatgtctggctctagctatcccgcccctaactccgcccatcccgcccctaactccgcccagttccgcccattctccgccccatggctgactaattttttttatttatgcagaggccgaggccgcctcggcctctgagctattccagaagtagtgaggaggcttttttggaggccgctagcgtcgaccattacttattgttttagctgtcctcatgaatgtcttttcactacccatttgcttatcctgcatctctcagccttgactccactcagttctcttgcttagagataccacctttcccctgaagtgttccttccatgttttacggcgagatggtttctcctcgcctggccactcagccttagttgtctctgttgtcttatagaggtctacttgaagaaggaaaaacagggggcatggtttgactgtcctgtgagcccttcttccctgcctcccccactcacagtgacccggaatccctcgacatggcagtctagcactagtgcggccgcagatctgcttcctcgctcactgactcgctgcgctcggtcgttcggctgcggcgagcggtatcagctcactcaaaggcggtaatacggttatccacagaatcaggggataacgcaggaaagaacatgtgagcaaaaggccagcaaaaggccaggaaccgtaaaaa

SEQ ID NO: 14 - DNA, 4484 bp, synthetic construct
  misc_feature 1..4484: note = pAAV-MCS-CBH-WPRE
  source 1..4484: mol_type = other DNA
acatgtgagcaaaaggccagcaaaaggccaggaaccgtaaaaaggccgcgttgctggcgtttttccataggctccgcccccctgacgagcatcacaaaaatcgacgctcaagtcagaggtggcgaaacccgacaggactataaagataccaggcgtttccccctggaagctccctcgtgcgctctcctgttccgaccctgccgcttaccggatacctgtccgcctttctcccttcgggaagcgtggcgctttctcatagctcacgctgtaggtatctcagttcggtgtaggtcgttcgctccaagctgggctgtgtgcacgaaccccccgttcagcccgaccgctgcgccttatccggtaactatcgtcttgagtccaacccggtaagacacgacttatcgccactggcagcagccactggtaacaggattagcagagcgaggtatgtaggcggtgctacagagttcttgaagtggtggcctaactacggctacactagaaggacagtatttggtatctgcgctctgctgaagccagttaccttcggaaaaagagttggtagctcttgatccggcaaacaaaccaccgctggtagcggtggtttttttgtttgcaagcagcagattacgcgcagaaaaaaaggatctcaagaagatcctttgatcttttctacggggtctgacgctcagtggaacgaaaactcacgttaagggattttggtcatgagattatcaaaaaggatcttcacctagatccttttaaattaaaaatgaagttttaaatcaatctaaagtatatatgagtaaacttggtctgacagttaccaatgcttaatcagtgaggcacctatctcagcgatctgtctatttcgttcatccatagttgcctgactccccgtcgtgtagataactacgatacgggagggcttaccatctggccccagtgctgcaatgataccgcgagacccacgctcaccggctccagatttatcagcaataaaccagccagccggaagggccgagcgcagaagtggtcctgcaactttatccgcctccatccagtctattaattgttgccgggaagctagagtaagtagttcgccagttaatagtttgcgcaacgttgttgccattgctacaggcatcgtggtgtcacgctcgtcgtttggtatggcttcattcagctccggttcccaacgatcaaggcgagttacatgatcccccatgttgtgcaaaaaagcggttagctccttcggtcctccgatcgttgtcagaagtaagttggccgcagtgttatcactcatggttatggcagcactgcataattctcttactgtcatgccatccgtaagatgcttttctgtgactggtgagtactcaaccaagtcattctgagaatagtgtatgcggcgaccgagttgctcttgcccggcgtcaatacgggataataccgcgccacatagcagaactttaaaagtgctcatcattggaaaacgttcttcggggcgaaaactctcaaggatcttaccgctgttgagatccagttcgatgtaacccactcgtgcacccaactgatcttcagcatcttttactttcaccagcgtttctgggtgagcaaaaacaggaaggcaaaatgccgcaaaaaagggaataagggcgacacggaaatgttgaatactcatactcttcctttttcaatattattgaagcatttatcagggttattgtctcatgagcggatacatatttgaatgtatttagaaaaataaacaaataggggttccgcgcacatttccccgaaaagtgccacctgacgtctaagaaaccattattatcatgacattaacctataaaaataggcgtatcacgaggccctttcgtctcgcgcgtttcggtgatgacggtgaaaacctctgacacatgcagctcccggagacggtcacagcttgtctgtaagcggatgccgggagcagacaagcccgtcagggcgcgtcagcgggtgttggcgggtgtcggggctggcttaactatgcggcatcagagcagattgtactgagagtgcaccataaaattgtaaacgttaatattttgttaaaattcgcgttaaatttttgttaaatcagctcattttttaaccaataggccgaaatcggcaaaatcccttataaatcaaaagaatagcccgagatagggttgagtgttgttccagtttggaacaagagtccactattaaagaacgtggactccaacgtcaaagggcgaaaaaccgtctatcagggcgatggcccactacgtgaaccatcacccaaatcaagttttttggggtcgaggtgccgtaaagcactaaatcggaaccctaaagggagcccccgatttagagcttgacggggaaagccggcgaacgtggcgagaaaggaagggaagaaagcgaaaggagcgggcgctagggcgctggcaagtgtagcggtcacgctgcgcgtaaccaccacacccgccgcgcttaatgcgccgctacagggcgcgtactatggttgctttgacgtatgcggtgtgaaataccgcacagatgcgtaaggagaaaataccgcatcaggcgcccctgcaggcagctgcgcgctcgctcgctcactgaggccgcccgggcaaagcccgggcgtcgggcgacctttggtcgcccggcctcagtgagcgagcgagcgcgcagagagggagtggccaactccatcactaggggttcctacgcgtcgttacataacttacggtaaatggcccgcctggctgaccgcccaacgacccccgcccattgacgtcaataatgacgtatgttcccatagtaacgccaatagggactttccattgacgtcaatgggtggagtatttacggtaaactgcccacttggcagtacatcaagtgtatcatatgccaagtacgccccctattgacgtcaatgacggtaaatggcccgcctggcattatgcccagtacatgaccttatgggactttcctacttggcagtacatctacgtattagtcatcgctattaccatggtcgaggtgagccccacgttctgcttcactctccccatctcccccccctccccacccccaattttgtatttatttattttttaattattttgtgcagcgatgggggcggggggggggggggggcgcgcgccaggcggggcggggcggggcgaggggcggggcggggcgaggcggagaggtgcggcggcagccaatcagagcggcgcgctccgaaagtttccttttatggcgaggcggcggcggcggcggccctataaaaagcgaagcgcgcggcgggcgggagtcgctgcgacgctgccttcgccccgtgccccgctccgccgccgcctcgcgccgcccgccccggctctgactgaccgcgttactcccacaggtgagcgggcgggacggcccttctcctccgggctgtaattagctgagcaagaggtaagggtttaagggatggttggttggtggggtattaatgtttaattacctggagcacctgcctgaaatcactttttttcaggtaccggtcgtcgacaatcaacctctggattacaaaatttgtgaaagattgactggtattcttaactatgttgctccttttacgctatgtggatacgctgctttaatgcctttgtatcatgctattgcttcccgtatggctttcattttctcctccttgtataaatcctggttgctgtctctttatgaggagttgtggcccgttgtcaggcaacgtggcgtggtgtgcactgtgtttgctgacgcaacccccactggttggggcattgccaccacctgtcagctcctttccgggactttcgctttccccctccctattgccacggcggaactcatcgccgcctgccttgcccgctgctggacaggggctcggctgttgggcactgacaattccgtggtgttgtcggggaagctgacgtcctttccatggctgctcgcctgtgttgccacctggattctgcgcgggacgtccttctgctacgtcccttcggccctcaatccagcggaccttccttcccgcggcctgctgccggctctgcggcctcttccgcgtcttcgccttcgccctcagacgagtcggatctccctttgggccgcctccccgcgaattcgtttatttgtgaaatttgtgatgctattgctttatttgtaaccatctagctttatttgtgaaatttgtgatgctattgctttatttgtaaccattataagctgcaataaacaagttaacaacaacaattgcattcattttatgtttcaggttcagggggagatgtgggaggttttttaaagtttaaacaggaacccctagtgatggagttggccactccctctctgcgcgctcgctcgctcactgaggccgggcgaccaaaggtcgcccgacgcccgggcggcctcagtgagcgagcgagcgcgcagctgcctgcagg

SEQ ID NO: 15 - DNA, 6149 bp, synthetic construct
  misc_feature 1..6149: note = pAAV-CBH-KL-BsHIV01-02-WPRE
  source 1..6149: mol_type = other DNA
acatgtgagcaaaaggccagcaaaaggccaggaaccgtaaaaaggccgcgttgctggcgtttttccataggctccgcccccctgacgagcatcacaaaaatcgacgctcaagtcagaggtggcgaaacccgacaggactataaagataccaggcgtttccccctggaagctccctcgtgcgctctcctgttccgaccctgccgcttaccggatacctgtccgcctttctcccttcgggaagcgtggcgctttctcatagctcacgctgtaggtatctcagttcggtgtaggtcgttcgctccaagctgggctgtgtgcacgaaccccccgttcagcccgaccgctgcgccttatccggtaactatcgtcttgagtccaacccggtaagacacgacttatcgccactggcagcagccactggtaacaggattagcagagcgaggtatgtaggcggtgctacagagttcttgaagtggtggcctaactacggctacactagaaggacagtatttggtatctgcgctctgctgaagccagttaccttcggaaaaagagttggtagctcttgatccggcaaacaaaccaccgctggtagcggtggtttttttgtttgcaagcagcagattacgcgcagaaaaaaaggatctcaagaagatcctttgatcttttctacggggtctgacgctcagtggaacgaaaactcacgttaagggattttggtcatgagattatcaaaaaggatcttcacctagatccttttaaattaaaaatgaagttttaaatcaatctaaagtatatatgagtaaacttggtctgacagttaccaatgcttaatcagtgaggcacctatctcagcgatctgtctatttcgttcatccatagttgcctgactccccgtcgtgtagataactacgatacgggagggcttaccatctggccccagtgctgcaatgataccgcgagacccacgctcaccggctccagatttatcagcaataaaccagccagccggaagggccgagcgcagaagtggtcctgcaactttatccgcctccatccagtctattaattgttgccgggaagctagagtaagtagttcgccagttaatagtttgcgcaacgttgttgccattgctacaggcatcgtggtgtcacgctcgtcgtttggtatggcttcattcagctccggttcccaacgatcaaggcgagttacatgatcccccatgttgtgcaaaaaagcggttagctccttcggtcctccgatcgttgtcagaagtaagttggccgcagtgttatcactcatggttatggcagcactgcataattctcttactgtcatgccatccgtaagatgcttttctgtgactggtgagtactcaaccaagtcattctgagaatagtgtatgcggcgaccgagttgctcttgcccggcgtcaatacgggataataccgcgccacatagcagaactttaaaagtgctcatcattggaaaacgttcttcggggcgaaaactctcaaggatcttaccgctgttgagatccagttcgatgtaacccactcgtgcacccaactgatcttcagcatcttttactttcaccagcgtttctgggtgagcaaaaacaggaaggcaaaatgccgcaaaaaagggaataagggcgacacggaaatgttgaatactcatactcttcctttttcaatattattgaagcatttatcagggttattgtctcatgagcggatacatatttgaatgtatttagaaaaataaacaaataggggttccgcgcacatttccccgaaaagtgccacctgacgtctaagaaaccattattatcatgacattaacctataaaaataggcgtatcacgaggccctttcgtctcgcgcgtttcggtgatgacggtgaaaacctctgacacatgcagctcccggagacggtcacagcttgtctgtaagcggatgccgggagcagacaagcccgtcagggcgcgtcagcgggtgttggcgggtgtcggggctggcttaactatgcggcatcagagcagattgtactgagagtgcaccataaaattgtaaacgttaatattttgttaaaattcgcgttaaatttttgttaaatcagctcattttttaaccaataggccgaaatcggcaaaatcccttataaatcaaaagaatagcccgagatagggttgagtgttgttccagtttggaacaagagtccactattaaagaacgtggactccaacgtcaaagggcgaaaaaccgtctatcagggcgatggcccactacgtgaaccatcacccaaatcaagttttttggggtcgaggtgccgtaaagcactaaatcggaaccctaaagggagcccccgatttagagcttgacggggaaagccggcgaacgtggcgagaaaggaagggaagaaagcgaaaggagcgggcgctagggcgctggcaagtgtagcggtcacgctgcgcgtaaccaccacacccgccgcgcttaatgcgccgctacagggcgcgtactatggttgctttgacgtatgcggtgtgaaataccgcacagatgcgtaaggagaaaataccgcatcaggcgcccctgcaggcagctgcgcgctcgctcgctcactgaggccgcccgggcaaagcccgggcgtcgggcgacctttggtcgcccggcctcagtgagcgagcgagcgcgcagagagggagtggccaactccatcactaggggttcctacgcgtcgttacataacttacggtaaatggcccgcctggctgaccgcccaacgacccccgcccattgacgtcaataatgacgtatgttcccatagtaacgccaatagggactttccattgacgtcaatgggtggagtatttacggtaaactgcccacttggcagtacatcaagtgtatcatatgccaagtacgccccctattgacgtcaatgacggtaaatggcccgcctggcattatgcccagtacatgaccttatgggactttcctacttggcagtacatctacgtattagtcatcgctattaccatggtcgaggtgagccccacgttctgcttcactctccccatctcccccccctccccacccccaattttgtatttatttattttttaattattttgtgcagcgatgggggcggggggggggggggggcgcgcgccaggcggggcggggcggggcgaggggcggggcggggcgaggcggagaggtgcggcggcagccaatcagagcggcgcgctccgaaagtttccttttatggcgaggcggcggcggcggcggccctataaaaagcgaagcgcgcggcgggcgggagtcgctgcgacgctgccttcgccccgtgccccgctccgccgccgcctcgcgccgcccgccccggctctgactgaccgcgttactcccacaggtgagcgggcgggacggcccttctcctccgggctgtaattagctgagcaagaggtaagggtttaagggatggttggttggtggggtattaatgtttaattacctggagcacctgcctgaaatcactttttttcaggtaccggtcgccaccatggcgagacccctgtgcacattacttctgttgatggctaccctggcaggcgccctcgccagcgagctgacacaggaccctgccgtgtccgtggccctgaagcagaccgtgacaatcacctgcagaggcgattccctgagatcccactacgcctcctggtaccagaagaagcctggccaggcccccgtgctgctgttttacggcaagaataaccgccccagcggcatccccgatagattttccggcagcgcctccggcaacagagccagcctgacaatcaccggcgcccaggccgaggacgaggctgattactactgcagctccagagataagagcggcagcagactgtccgtgtttggcggcggcaccaagctgaccgtgctcggaggaggaggaagcggaggaggaggctcaggcggcggcggctctgaggtgaggctgagagagtccggcggcggcctggtgaagcccggaggatctctgaggctgtcctgctccgcctccggcttcgattttgacaatgcctggatgacctgggtgagacagccccctggcaagggcctggagtgggtgggaaggatcacaggccccggcgagggctggtccgtggattacgccgagtccgtgaagggcaggttcacaatctccagggataacaccaagaacaccctgtacctggagatgaacaacgtgaggacagaggataccggctactacttttgcgccagaacaggcaagtactacgacttttggttcggctacccccctggcgaggagtacttccaggattggggccagggcaccctggtcattgtgtccagcggcggcggcggcagtggcggcggcggaagcggcggcggcggctctggcggcggcggcagcggcggcggcggctccgacatcgtgatgacccagtctcctgatagcctggccgtgagcctgggcgagagagtgacaatgaactgtaagtctagccagagcctgctgtactccaccaaccagaagaattacctggcctggtatcagcagaagcctggccagtccccaaagctgctgatctattgggcatctacaagggagagcggagtgccagacagattcagcggatccggatctggaaccgacttcaccctgacaatctcctctgtgcaggccgaggacgtggccgtgtactattgccagcagtactatagctacaggacattcggcggcggcaccaagctggagatcaagcgcaccgtggccggaggaggaggatctggcggaggagggtccggcggcggcggctcccaggtgcagctgcagcagagcggaccagaggtggtgaagcctggagcctccgtgaagatgtcttgtaaggccagcggctacaccttcacatcctatgtgatccactgggtgaggcagaagccaggacagggactggactggatcggctacatcaacccttataatgatggcaccgactacgatgagaagtttaagggcaaggccaccctgacatccgataccagcacatccaccgcctatatggagctgagctccctgcggtctgaggacacagccgtgtactattgcgccagagagaaggataactacgcaaccggagcatggttcgcatattggggacagggtaccctggtcaccgtgtctagctaggtcgacaatcaacctctggattacaaaatttgtgaaagattgactggtattcttaactatgttgctccttttacgctatgtggatacgctgctttaatgcctttgtatcatgctattgcttcccgtatggctttcattttctcctccttgtataaatcctggttgctgtctctttatgaggagttgtggcccgttgtcaggcaacgtggcgtggtgtgcactgtgtttgctgacgcaacccccactggttggggcattgccaccacctgtcagctcctttccgggactttcgctttccccctccctattgccacggcggaactcatcgccgcctgccttgcccgctgctggacaggggctcggctgttgggcactgacaattccgtggtgttgtcggggaagctgacgtcctttccatggctgctcgcctgtgttgccacctggattctgcgcgggacgtccttctgctacgtcccttcggccctcaatccagcggaccttccttcccgcggcctgctgccggctctgcggcctcttccgcgtcttcgccttcgccctcagacgagtcggatctccctttgggccgcctccccgcgaattcgtttatttgtgaaatttgtgatgctattgctttatttgtaaccatctagctttatttgtgaaatttgtgatgctattgctttatttgtaaccattataagctgcaataaacaagttaacaacaacaattgcattcattttatgtttcaggttcagggggagatgtgggaggttttttaaagtttaaacaggaacccctagtgatggagttggccactccctctctgcgcgctcgctcgctcactgaggccgggcgaccaaaggtcgcccgacgcccgggcggcctcagtgagcgagcgagcgcgcagctgcctgcagg

SEQ ID NO: 16 - DNA, 6311 bp, synthetic construct
  misc_feature 1..6311: note = pAAV-CBH-KL-BsHIV01-003-02-WPRE
  source 1..6311: mol_type = other DNA
acatgtgagcaaaaggccagcaaaaggccaggaaccgtaaaaaggccgcgttgctggcgtttttccataggctccgcccccctgacgagcatcacaaaaatcgacgctcaagtcagaggtggcgaaacccgacaggactataaagataccaggcgtttccccctggaagctccctcgtgcgctctcctgttccgaccctgccgcttaccggatacctgtccgcctttctcccttcgggaagcgtggcgctttctcatagctcacgctgtaggtatctcagttcggtgtaggtcgttcgctccaagctgggctgtgtgcacgaaccccccgttcagcccgaccgctgcgccttatccggtaactatcgtcttgagtccaacccggtaagacacgacttatcgccactggcagcagccactggtaacaggattagcagagcgaggtatgtaggcggtgctacagagttcttgaagtggtggcctaactacggctacactagaaggacagtatttggtatctgcgctctgctgaagccagttaccttcggaaaaagagttggtagctcttgatccggcaaacaaaccaccgctggtagcggtggtttttttgtttgcaagcagcagattacgcgcagaaaaaaaggatctcaagaagatcctttgatcttttctacggggtctgacgctcagtggaacgaaaactcacgttaagggattttggtcatgagattatcaaaaaggatcttcacctagatccttttaaattaaaaatgaagttttaaatcaatctaaagtatatatgagtaaacttggtctgacagttaccaatgcttaatcagtgaggcacctatctcagcgatctgtctatttcgttcatccatagttgcctgactccccgtcgtgtagataactacgatacgggagggcttaccatctggccccagtgctgcaatgataccgcgagacccacgctcaccggctccagatttatcagcaataaaccagccagccggaagggccgagcgcagaagtggtcctgcaactttatccgcctccatccagtctattaattgttgccgggaagctagagtaagtagttcgccagttaatagtttgcgcaacgttgttgccattgctacaggcatcgtggtgtcacgctcgtcgtttggtatggcttcattcagctccggttcccaacgatcaaggcgagttacatgatcccccatgttgtgcaaaaaagcggttagctccttcggtcctccgatcgttgtcagaagtaagttggccgcagtgttatcactcatggttatggcagcactgcataattctcttactgtcatgccatccgtaagatgcttttctgtgactggtgagtactcaaccaagtcattctgagaatagtgtatgcggcgaccgagttgctcttgcccggcgtcaatacgggataataccgcgccacatagcagaactttaaaagtgctcatcattggaaaacgttcttcggggcgaaaactctcaaggatcttaccgctgttgagatccagttcgatgtaacccactcgtgcacccaactgatcttcagcatcttttactttcaccagcgtttctgggtgagcaaaaacaggaaggcaaaatgccgcaaaaaagggaataagggcgacacggaaatgttgaatactcatactcttcctttttcaatattattgaagcatttatcagggttattgtctcatgagcggatacatatttgaatgtatttagaaaaataaacaaataggggttccgcgcacatttccccgaaaagtgccacctgacgtctaagaaaccattattatcatgacattaacctataaaaataggcgtatcacgaggccctttcgtctcgcgcgtttcggtgatgacggtgaaaacctctgacacatgcagctcccggagacggtcacagcttgtctgtaagcggatgccgggagcagacaagcccgtcagggcgcgtcagcgggtgttggcgggtgtcggggctggcttaactatgcggcatcagagcagattgtactgagagtgcaccataaaattgtaaacgttaatattttgttaaaattcgcgttaaatttttgttaaatcagctcattttttaaccaataggccgaaatcggcaaaatcccttataaatcaaaagaatagcccgagatagggttgagtgttgttccagtttggaacaagagtccactattaaagaacgtggactccaacgtcaaagggcgaaaaaccgtctatcagggcgatggcccactacgtgaaccatcacccaaatcaagttttttggggtcgaggtgccgtaaagcactaaatcggaaccctaaagggagcccccgatttagagcttgacggggaaagccggcgaacgtggcgagaaaggaagggaagaaagcgaaaggagcgggcgctagggcgctggcaagtgtagcggtcacgctgcgcgtaaccaccacacccgccgcgcttaatgcgccgctacagggcgcgtactatggttgctttgacgtatgcggtgtgaaataccgcacagatgcgtaaggagaaaataccgcatcaggcgcccctgcaggcagctgcgcgctcgctcgctcactgaggccgcccgggcaaagcccgggcgtcgggcgacctttggtcgcccggcctcagtgagcgagcgagcgcgcagagagggagtggccaactccatcactaggggttcctacgcgtcgttacataacttacggtaaatggcccgcctggctgaccgcccaacgacccccgcccattgacgtcaataatgacgtatgttcccatagtaacgccaatagggactttccattgacgtcaatgggtggagtatttacggtaaactgcccacttggcagtacatcaagtgtatcatatgccaagtacgccccctattgacgtcaatgacggtaaatggcccgcctggcattatgcccagtacatgaccttatgggactttcctacttggcagtacatctacgtattagtcatcgctattaccatggtcgaggtgagccccacgttctgcttcactctccccatctcccccccctccccacccccaattttgtatttatttattttttaattattttgtgcagcgatgggggcggggggggggggggggcgcgcgccaggcggggcggggcggggcgaggggcggggcggggcgaggcggagaggtgcggcggcagccaatcagagcggcgcgctccgaaagtttccttttatggcgaggcggcggcggcggcggccctataaaaagcgaagcgcgcggcgggcgggagtcgctgcgacgctgccttcgccccgtgccccgctccgccgccgcctcgcgccgcccgccccggctctgactgaccgcgttactcccacaggtgagcgggcgggacggcccttctcctccgggctgtaattagctgagcaagaggtaagggtttaagggatggttggttggtggggtattaatgtttaattacctggagcacctgcctgaaatcactttttttcaggtaccggtcgccaccatggcgagacccctgtgcacattacttctgttgatggctaccctggcaggcgccctcgccagcgagctgacacaggaccctgccgtgtccgtggccctgaagcagaccgtgacaatcacctgcagaggcgattccctgagatcccactacgcctcctggtaccagaagaagcctggccaggcccccgtgctgctgttttacggcaagaataaccgccccagcggcatccccgatagattttccggcagcgcctccggcaacagagccagcctgacaatcaccggcgcccaggccgaggacgaggctgattactactgcagctccagagataagagcggcagcagactgtccgtgtttggcggcggcaccaagctgaccgtgctcggaggaggaggaagcggaggaggaggctcaggcggcggcggctctgaggtgaggctgagagagtccggcggcggcctggtgaagcccggaggatctctgaggctgtcctgctccgcctccggcttcgattttgacaatgcctggatgacctgggtgagacagccccctggcaagggcctggagtgggtgggaaggatcacaggccccggcgagggctggtccgtggattacgccgagtccgtgaagggcaggttcacaatctccagggataacaccaagaacaccctgtacctggagatgaacaacgtgaggacagaggataccggctactacttttgcgccagaacaggcaagtactacgacttttggttcggctacccccctggcgaggagtacttccaggattggggccagggcaccctggtcattgtgtccagcggcggcggcggcagtggcggcggcggaagcggcggcggcggctctggcggcggcggcagcggcggcggcggctccgacatcgtgatgacccagtctcctgatagcctggccgtgagcctgggcgagagagtgacaatgaactgtaagtctagccagagcctgctgtactccaccaaccagaagaattacctggcctggtatcagcagaagcctggccagtccccaaagctgctgatctattgggcatctacaagggagagcggagtgccagacagattcagcggatccggatctggaaccgacttcaccctgacaatctcctctgtgcaggccgaggacgtggccgtgtactattgccagcagtactatagctacaggacattcggcggcggcaccaagctggagatcaagcgcaccgtggccggaggaggaggatctggcggaggagggtccggcggcggcggctcccaggtgcagctgcagcagagcggaccagaggtggtgaagcctggagcctccgtgaagatgtcttgtaaggccagcggctacaccttcacatcctatgtgatccactgggtgaggcagaagccaggacagggactggactggatcggctacatcaacccttataatgatggcaccgactacgatgagaagtttaagggcaaggccaccctgacatccgataccagcacatccaccgcctatatggagctgagctccctgcggtctgaggacacagccgtgtactattgcgccagagagaaggataactacgcaaccggagcatggttcgcatattggggacagggtaccctggtcaccgtgtctagcggcggaggaggaagcggaggaggcggctctggcggaggaggttccggaggaggcggaagcggcggaggaggctcttgggagcagaagatcgaggagctgctgaagaaggccgaggagcagcagaagaagaatgaggaggagctgaagaagctggagaagtaggtcgacgacaatcaacctctggattacaaaatttgtgaaagattgactggtattcttaactatgttgctccttttacgctatgtggatacgctgctttaatgcctttgtatcatgctattgcttcccgtatggctttcattttctcctccttgtataaatcctggttgctgtctctttatgaggagttgtggcccgttgtcaggcaacgtggcgtggtgtgcactgtgtttgctgacgcaacccccactggttggggcattgccaccacctgtcagctcctttccgggactttcgctttccccctccctattgccacggcggaactcatcgccgcctgccttgcccgctgctggacaggggctcggctgttgggcactgacaattccgtggtgttgtcggggaagctgacgtcctttccatggctgctcgcctgtgttgccacctggattctgcgcgggacgtccttctgctacgtcccttcggccctcaatccagcggaccttccttcccgcggcctgctgccggctctgcggcctcttccgcgtcttcgccttcgccctcagacgagtcggatctccctttgggccgcctccccgcgaattcgtttatttgtgaaatttgtgatgctattgctttatttgtaaccatctagctttatttgtgaaatttgtgatgctattgctttatttgtaaccattataagctgcaataaacaagttaacaacaacaattgcattcattttatgtttcaggttcagggggagatgtgggaggttttttaaagtttaaacaggaacccctagtgatggagttggccactccctctctgcgcgctcgctcgctcactgaggccgggcgaccaaaggtcgcccgacgcccgggcggcctcagtgagcgagcgagcgcgcagctgcctgcagg

SEQ ID NO: 17 - DNA, 5612 bp, synthetic construct
  misc_feature 1..5612: note = pKL-Kan-Vsvg
  source 1..5612: mol_type = other DNA
ggccgcgttgctggcgtttttccataggctccgcccccctgacgagcatcacaaaaatcgacgctcaagtcagaggtggcgaaacccgacaggactataaagataccaggcgtttccccctggaagctccctcgtgcgctctcctgttccgaccctgccgcttaccggatacctgtccgcctttctcccttcgggaagcgtggcgctttctcatagctcacgctgtaggtatctcagttcggtgtaggtcgttcgctccaagctgggctgtgtgcacgaaccccccgttcagcccgaccgctgcgccttatccggtaactatcgtcttgagtccaacccggtaagacacgacttatcgccactggcagcagccactggtaacaggattagcagagcgaggtatgtaggcggtgctacagagttcttgaagtggtggcctaactacggctacactagaagaacagtatttggtatctgcgctctgctgaagccagttaccttcggaaaaagagttggtagctcttgatccggcaaacaaaccaccgctggtagcggtggtttttttgtttgcaagcagcagattacgcgcagaaaaaaaggatctcaagaagatcctttgatcttttctacggggtctgacgctcagtggaacgaaaactcacgttaagggattttggtcatgaagcgcttttgaagctcggatccgaacaaacgacccaacacccgtgcgttttattctgtctttttattgccgatcccctcagaagaactcgtcaagaaggcgatagaaggcgatgcgctgcgaatcgggagcggcgataccgtaaagcacgaggaagcggtcagcccattcgccgccaagctcttcagcaatatcacgggtagccaacgctatgtcctgatagcggtccgccacacccagccggccacagtcgatgaatccagaaaagcggccattttccaccatgatattcggcaagcaggcatcgccatgggtcacgacgagatcctcgccgtcgggcatgctcgccttgagcctggcgaacagttcggctggcgcgagcccctgatgctcttcgtccagatcatcctgatcgacaagaccggcttccatccgagtacgtgctcgctcgatgcgatgtttcgcttggtggtcgaatgggcaggtagccggatcaagcgtatgcagccgccgcattgcatcagccatgatggatactttctcggcaggagcaaggtgagatgacaggagatcctgccccggcacttcgcccaatagcagccagtcccttcccgcttcagtgacaacgtcgagcacagctgcgcaaggaacgcccgtcgtggccagccacgatagccgcgctgcctcgtcttgcagttcattcagggcaccggacaggtcggtcttgacaaaaagaaccgggcgcccctgcgctgacagccggaacacggcggcatcagagcagccgattgtctgttgtgcccagtcatagccgaatagcctctccacccaagcggccggagaacctgcgtgcaatccatcttgttcaatcatgcgaaacgatcctcatcctgtctcttgatcagagcttgatcccctgcgccatcagatccttggcggcaagaaagccatccagtttactttgcagggcttcccaaccttaccagaggcctgcgccgcggccagctggctagcaattcccgggttaactctagagacattgattattgactagttattaatagtaatcaattacggggtcattagttcatagcccatatatggagttccgcgttacataacttacggtaaatggcccgcctggctgaccgcccaacgacccccgcccattgacgtcaataatgacgtatgttcccatagtaacgccaatagggactttccattgacgtcaatgggtggagtatttacggtaaactgcccacttggcagtacatcaagtgtatcatatgccaagtacgccccctattgacgtcaatgacggtaaatggcccgcctggcattatgcccagtacatgaccttatgggactttcctacttggcagtacatctacgtattagtcatcgctattaccatggtgatgcggttttggcagtacatcaatgggcgtggatagcggtttgactcacggggatttccaagtctccaccccattgacgtcaatgggagtttgttttggcaccaaaatcaacgggactttccaaaatgtcgtaacaactccgccccattgacgcaaatgggcggtaggcgtgtacggtgggaggtctatataagcagagctcgtttagtgaaccgtcagatcgcctggagacgccatccacgctgttttgacctccatagaagacaccgggaccgatccagcctcccctcgaagcttacatgtggtaccgagctcggatcctgagaacttcagggtgagtctatgggacccttgatgttttctttccccttcttttctatggttaagttcatgtcataggaaggggagaagtaacagggtacacatattgaccaaatcagggtaattttgcatttgtaattttaaaaaatgctttcttcttttaatatacttttttgtttatcttatttctaatactttccctaatctctttctttcagggcaataatgatacaatgtatcatgcctctttgcaccattctaaagaataacagtgataatttctgggttaaggcaatagcaatatttctgcatataaatatttctgcatataaattgtaactgatgtaagaggtttcatattgctaatagcagctacaatccagctaccattctgcttttattttatggttgggataaggctggattattctgagtccaagctaggcccttttgctaatcatgttcatacctcttatcttcctcccacagctcctgggcaacgtgctggtctgtgtgctggcccatcactttggcaaagcacgtgagatctgaattctgacactatgaagtgccttttgtacttagcctttttattcattggggtgaattgcaagttcaccatagtttttccacacaaccaaaaaggaaactggaaaaatgttccttctaattaccattattgcccgtcaagctcagatttaaattggcataatgacttaataggcacagccttacaagtcaaaatgcccaagagtcacaaggctattcaagcagacggttggatgtgtcatgcttccaaatgggtcactacttgtgatttccgctggtatggaccgaagtatataacacattccatccgatccttcactccatctgtagaacaatgcaaggaaagcattgaacaaacgaaacaaggaacttggctgaatccaggcttccctcctcaaagttgtggatatgcaactgtgacggatgccgaagcagtgattgtccaggtgactcctcaccatgtgctggttgatgaatacacaggagaatgggttgattcacagttcatcaacggaaaatgcagcaattacatatgccccactgtccataactctacaacctggcattctgactataaggtcaaagggctatgtgattctaacctcatttccatggacatcaccttcttctcagaggacggagagctatcatccctgggaaaggagggcacagggttcagaagtaactactttgcttatgaaactggaggcaaggcctgcaaaatgcaatactgcaagcattggggagtcagactcccatcaggtgtctggttcgagatggctgataaggatctctttgctgcagccagattccctgaatgcccagaagggtcaagtatctctgctccatctcagacctcagtggatgtaagtctaattcaggacgttgagaggatcttggattattccctctgccaagaaacctggagcaaaatcagagcgggtcttccaatctctccagtggatctcagctatcttgctcctaaaaacccaggaaccggtcctgctttcaccataatcaatggtaccctaaaatactttgagaccagatacatcagagtcgatattgctgctccaatcctctcaagaatggtcggaatgatcagtggaactaccacagaaagggaactgtgggatgactgggcaccatatgaagacgtggaaattggacccaatggagttctgaggaccagttcaggatataagtttcctttatacatgattggacatggtatgttggactccgatcttcatcttagctcaaaggctcaggtgttcgaacatcctcacattcaagacgctgcttcgcaacttcctgatgatgagagtttattttttggtgatactgggctatccaaaaatccaatcgagcttgtagaaggttggttcagtagttggaaaagctctattgcctcttttttctttatcatagggttaatcattggactattcttggttctccgagttggtatccatctttgcattaaattaaagcacaccaagaaaagacagatttatacagacatagagatgaaccgacttggaaagtaactcaaatcctgcacaacagattcttcatgtttggaccaaatcaacttgtgataccatgctcaaagaggcctcaattatatttgagtttttaatttttatgaaaaaaaaaaaaaaaaacggaattcaccccaccagtgcaggctgcctatcagaaagtggtggctggtgtggctaatgccctggcccacaagtatcactaagctcgctttcttgctgtccaatttctattaaaggttcctttgttccctaagtccaactactaaactgggggatattatgaagggccttgagcatctggattctgcctaataaaaaacatttattttcattgcaatgatgtatttaaattatttctgaatattttactaaaaagggaatgtgggaggtcagtgcatttaaaacataaagaaatgaagagctagttcaaaccttgggaaaatacactatatcttaaactccatgaaagaaggtgaggctgcaaacagctaatgcacattggcaacagcccctgatgcctatgccttattcatccctcagaaaaggattcaagtagaggcttgatttggaggttaaagttttgctatgctgtattttagtcgaccattacttattgttttagctgtcctcatgaatgtcttttcactacccatttgcttatcctgcatctctcagccttgactccactcagttctcttgcttagagataccacctttcccctgaagtgttccttccatgttttacggcgagatggtttctcctcgcctggccactcagccttagttgtctctgttgtcttatagaggtctacttgaagaaggaaaaacagggggcatggtttgactgtcctgtgagcccttcttccctgcctcccccactcacagtgacccggaatccctcgacatggcagtctagcactagtgcggccgcagatctgcttcctcgctcactgactcgctgcgctcggtcgttcggctgcggcgagcggtatcagctcactcaaaggcggtaatacggttatccacagaatcaggggataacgcaggaaagaacatgtgagcaaaaggccagcaaaaggccaggaaccgtaaaaa

SEQ ID NO: 18 - DNA, 3387 bp, synthetic construct
  misc_feature 1..3387: note = pKL-Kan-Rev
  source 1..3387: mol_type = other DNA
ggccgcgttgctggcgtttttccataggctccgcccccctgacgagcatcacaaaaatcgacgctcaagtcagaggtggcgaaacccgacaggactataaagataccaggcgtttccccctggaagctccctcgtgcgctctcctgttccgaccctgccgcttaccggatacctgtccgcctttctcccttcgggaagcgtggcgctttctcatagctcacgctgtaggtatctcagttcggtgtaggtcgttcgctccaagctgggctgtgtgcacgaaccccccgttcagcccgaccgctgcgccttatccggtaactatcgtcttgagtccaacccggtaagacacgacttatcgccactggcagcagccactggtaacaggattagcagagcgaggtatgtaggcggtgctacagagttcttgaagtggtggcctaactacggctacactagaagaacagtatttggtatctgcgctctgctgaagccagttaccttcggaaaaagagttggtagctcttgatccggcaaacaaaccaccgctggtagcggtggtttttttgtttgcaagcagcagattacgcgcagaaaaaaaggatctcaagaagatcctttgatcttttctacggggtctgacgctcagtggaacgaaaactcacgttaagggattttggtcatgaagcgcttttgaagctcggatccgaacaaacgacccaacacccgtgcgttttattctgtctttttattgccgatcccctcagaagaactcgtcaagaaggcgatagaaggcgatgcgctgcgaatcgggagcggcgataccgtaaagcacgaggaagcggtcagcccattcgccgccaagctcttcagcaatatcacgggtagccaacgctatgtcctgatagcggtccgccacacccagccggccacagtcgatgaatccagaaaagcggccattttccaccatgatattcggcaagcaggcatcgccatgggtcacgacgagatcctcgccgtcgggcatgctcgccttgagcctggcgaacagttcggctggcgcgagcccctgatgctcttcgtccagatcatcctgatcgacaagaccggcttccatccgagtacgtgctcgctcgatgcgatgtttcgcttggtggtcgaatgggcaggtagccggatcaagcgtatgcagccgccgcattgcatcagccatgatggatactttctcggcaggagcaaggtgagatgacaggagatcctgccccggcacttcgcccaatagcagccagtcccttcccgcttcagtgacaacgtcgagcacagctgcgcaaggaacgcccgtcgtggccagccacgatagccgcgctgcctcgtcttgcagttcattcagggcaccggacaggtcggtcttgacaaaaagaaccgggcgcccctgcgctgacagccggaacacggcggcatcagagcagccgattgtctgttgtgcccagtcatagccgaatagcctctccacccaagcggccggagaacctgcgtgcaatccatcttgttcaatcatgcgaaacgatcctcatcctgtctcttgatcagagcttgatcccctgcgccatcagatccttggcggcaagaaagccatccagtttactttgcagggcttcccaaccttaccagaggcctgcgccgcggccagctggctagcaattcccgggttaactctagagaatgtagtcttatgcaatactcttgtagtcttgcaacatggtaacgatgagttagcaacatgccttacaaggagagaaaaagcaccgtgcatgccgattggtggaagtaaggtggtacgatcgtgccttattaggaaggcaacagacgggtctgacatggattggacgaaccactgaattccgcattgcagagatattgtatttaagtgcctagctcgatacaataaacgccatttgaccattcaccacattggtgtgcacctccaagctcgagctcgtttagtgaaccgtcagatcgcctggagacgccatccacgctgttttgacctccatagaagacaccgggaccgatccagcctcccctcgaagctagtcgattaggcatctcctatggcaggaagaagcggagacagcgacgaagacctcctcaaggcagtcagactcatcaagtttctctatcaaagcaacccacctcccaatcccgaggggacccgacaggcccgaaggaatagaagaagaaggtggagagagagacagagacagatccattcgattagtgaacggatccttagcacttatctgggacgatctgcggagcctgtgcctcttcagctaccaccgcttgagagacttactcttgattgtaacgaggattgtggaacttctgggacgcagggggtgggaagccctcaaatattggtggaatctcctacaatattggagtcaggagctaaagaatagtgctgttagcttgctcaatgccacagctatagcagtagctgaggggacagatagggttatagaagtagtacaagaagcttggcactggccgtcgttttacaacgtcgtgatctgagcctgggagatctctggctaactagggaacccactgcttaagcctcaataaagcttgccttgagtgcttcaagtagtgtgtgcccgtctgttgtgtgactctggtaactagagatcaggaaaaccctggcgttacccaacttaatcgccttgcagcacatccccctttcgccagctggcgtaatagcgaagaggcccgcaccgatcgcccttcccaacagttgcgcagcctgaatggcgaatggcgcctgatgcggtattttctccttacgcatctgtgcggtatttcacaccgcatacgtcaaagcaaccatagtgtcgaccattacttattgttttagctgtcctcatgaatgtcttttcactacccatttgcttatcctgcatctctcagccttgactccactcagttctcttgcttagagataccacctttcccctgaagtgttccttccatgttttacggcgagatggtttctcctcgcctggccactcagccttagttgtctctgttgtcttatagaggtctacttgaagaaggaaaaacagggggcatggtttgactgtcctgtgagcccttcttccctgcctcccccactcacagtgacccggaatccctcgacatggcagtctagcactagtgcggccgcagatctgcttcctcgctcactgactcgctgcgctcggtcgttcggctgcggcgagcggtatcagctcactcaaaggcggtaatacggttatccacagaatcaggggataacgcaggaaagaacatgtgagcaaaaggccagcaaaaggccaggaaccgtaaaaa

SEQ ID NO: 19 - DNA, 9171 bp, synthetic construct
  misc_feature 1..9171: note = pKL-Kan-GagPol
  source 1..9171: mol_type = other DNA
ggccgcgttgctggcgtttttccataggctccgcccccctgacgagcatcacaaaaatcgacgctcaagtcagaggtggcgaaacccgacaggactataaagataccaggcgtttccccctggaagctccctcgtgcgctctcctgttccgaccctgccgcttaccggatacctgtccgcctttctcccttcgggaagcgtggcgctttctcatagctcacgctgtaggtatctcagttcggtgtaggtcgttcgctccaagctgggctgtgtgcacgaaccccccgttcagcccgaccgctgcgccttatccggtaactatcgtcttgagtccaacccggtaagacacgacttatcgccactggcagcagccactggtaacaggattagcagagcgaggtatgtaggcggtgctacagagttcttgaagtggtggcctaactacggctacactagaagaacagtatttggtatctgcgctctgctgaagccagttaccttcggaaaaagagttggtagctcttgatccggcaaacaaaccaccgctggtagcggtggtttttttgtttgcaagcagcagattacgcgcagaaaaaaaggatctcaagaagatcctttgatcttttctacggggtctgacgctcagtggaacgaaaactcacgttaagggattttggtcatgaagcgcttttgaagctcggatccgaacaaacgacccaacacccgtgcgttttattctgtctttttattgccgatcccctcagaagaactcgtcaagaaggcgatagaaggcgatgcgctgcgaatcgggagcggcgataccgtaaagcacgaggaagcggtcagcccattcgccgccaagctcttcagcaatatcacgggtagccaacgctatgtcctgatagcggtccgccacacccagccggccacagtcgatgaatccagaaaagcggccattttccaccatgatattcggcaagcaggcatcgccatgggtcacgacgagatcctcgccgtcgggcatgctcgccttgagcctggcgaacagttcggctggcgcgagcccctgatgctcttcgtccagatcatcctgatcgacaagaccggcttccatccgagtacgtgctcgctcgatgcgatgtttcgcttggtggtcgaatgggcaggtagccggatcaagcgtatgcagccgccgcattgcatcagccatgatggatactttctcggcaggagcaaggtgagatgacaggagatcctgccccggcacttcgcccaatagcagccagtcccttcccgcttcagtgacaacgtcgagcacagctgcgcaaggaacgcccgtcgtggccagccacgatagccgcgctgcctcgtcttgcagttcattcagggcaccggacaggtcggtcttgacaaaaagaaccgggcgcccctgcgctgacagccggaacacggcggcatcagagcagccgattgtctgttgtgcccagtcatagccgaatagcctctccacccaagcggccggagaacctgcgtgcaatccatcttgttcaatcatgcgaaacgatcctcatcctgtctcttgatcagagcttgatcccctgcgccatcagatccttggcggcaagaaagccatccagtttactttgcagggcttcccaaccttaccagaggcctgcgccgcggccagctggctagcaattcccgggttaactctagagacattgattattgactagttattaatagtaatcaattacggggtcattagttcatagcccatatatggagttccgcgttacataacttacggtaaatggcccgcctggctgaccgcccaacgacccccgcccattgacgtcaataatgacgtatgttcccatagtaacgccaatagggactttccattgacgtcaatgggtggagtatttacggtaaactgcccacttggcagtacatcaagtgtatcatatgccaagtacgccccctattgacgtcaatgacggtaaatggcccgcctggcattatgcccagtacatgaccttatgggactttcctacttggcagtacatctacgtattagtcatcgctattaccatggtgatgcggttttggcagtacatcaatgggcgtggatagcggtttgactcacggggatttccaagtctccaccccattgacgtcaatgggagtttgttttggcaccaaaatcaacgggactttccaaaatgtcgtaacaactccgccccattgacgcaaatgggcggtaggcgtgtacggtgggaggtctatataagcagagctcgtttagtgaaccgtcagatcgcctggagacgccatccacgctgttttgacctccatagaagacaccgggaccgatccagcctcccctcgaagcttacatgtggtaccgagctcggatcctgagaacttcagggtgagtctatgggacccttgatgttttctttccccttcttttctatggttaagttcatgtcataggaaggggagaagtaacagggtacacatattgaccaaatcagggtaattttgcatttgtaattttaaaaaatgctttcttcttttaatatacttttttgtttatcttatttctaatactttccctaatctctttctttcagggcaataatgatacaatgtatcatgcctctttgcaccattctaaagaataacagtgataatttctgggttaaggcaatagcaatatttctgcatataaatatttctgcatataaattgtaactgatgtaagaggtttcatattgctaatagcagctacaatccagctaccattctgcttttattttatggttgggataaggctggattattctgagtccaagctaggcccttttgctaatcatgttcatacctcttatcttcctcccacagctcctgggcaacgtgctggtctgtgtgctggcccatcactttggcaaagcacgtgagatctgaattcgagatctgccgccgccatgggtgcgagagcgtcagtattaagcgggggagaattagatcgatgggaaaaaattcggttaaggccagggggaaagaaaaaatataaattaaaacatatagtatgggcaagcagggagctagaacgattcgcagttaatcctggcctgttagaaacatcagaaggctgtagacaaatactgggacagctacaaccatcccttcagacaggatcagaagaacttagatcattatataatacagtagcaaccctctattgtgtgcatcaaaggatagagataaaagacaccaaggaagctttagacaagatagaggaagagcaaaacaaaagtaagaaaaaagcacagcaagcagcagctgacacaggacacagcaatcaggtcagccaaaattaccctatagtgcagaacatccaggggcaaatggtacatcaggccatatcacctagaactttaaatgcatgggtaaaagtagtagaagagaaggctttcagcccagaagtgatacccatgttttcagcattatcagaaggagccaccccacaagatttaaacaccatgctaaacacagtggggggacatcaagcagccatgcaaatgttaaaagagaccatcaatgaggaagctgcagaatgggatagagtgcatccagtgcatgcagggcctattgcaccaggccagatgagagaaccaaggggatcagacatcgctggaactactagtacccttcaggaacaaataggatggatgacacataatccacctatcccagtaggagaaatctataaaagatggataatcctgggattaaataaaatagtaagaatgtatagccctaccagcattctggacataagacaaggaccaaaggaaccctttagagactatgtagaccgattctataaaactctaagagccgagcaagcttcacaagaggtaaaaaattggatgacagaaaccttgttggtccaaaatgcgaacccagattgtaagactattttaaaagcattgggaccaggagcgacactagaagaaatgatgacagcatgtcagggagtggggggacccggccataaagcaagagttttggctgaagcaatgagccaagtaacaaatccagctaccataatgatacagaaaggcaattttaggaaccaaagaaagactgttaagtgtttcaattgtggcaaagaagggcacatagccaaaaattgcagggcccctaggaaaaagggctgttggaaatgtggaaaggaaggacaccaaatgaaagattgtactgagagacaggctaattttttagggaagatctggccttcccacaagggaaggccagggaattttcttcagagcagaccagagccaacagccccaccagaagagagcttcaggtttggggaagagacaacaactccctctcagaagcaggagccgatagacaaggaactgtatcctttagcttccctcagatcactctttggcagcgacccctcgtcacaataaagataggggggcaattaaaggaagctctattagatactggtgctgacgacacagtattagaagaaatgaatttgccaggaagatggaaaccaaaaatgatagggggaattggaggttttatcaaagtaagacagtatgatcagatactcatagaaatctgcggacataaagctataggtacagtattagtaggacctacacctgtcaacataattggaagaaatctgttgactcagattggctgcactttaaattttcccattagtcctattgagactgtaccagtaaaattaaagccaggaatggatggcccaaaagttaaacaatggccattgacagaagaaaaaataaaagcattagtagaaatttgtacagaaatggaaaaggaaggaaaaatttcaaaaattgggcctgaaaatccatacaatactccagtatttgccataaagaaaaaagacagtactaaatggagaaaattagtagatttcagagaacttaataagagaactcaagatttctgggaagttcaattaggaataccacatcctgcagggttaaaacagaaaaaatcagtaacagtactggatgtgggcgatgcatatttttcagttcccttagataaagacttcaggaagtatactgcatttaccatacctagtataaacaatgagacaccagggattagatatcagtacaatgtgcttccacagggatggaaaggatcaccagcaatattccagtgtagcatgacaaaaatcttagagccttttagaaaacaaaatccagacatagtcatctatcaatacatggatgatttgtatgtaggatctgacttagaaatagggcagcatagaacaaaaatagaggaactgagacaacatctgttgaggtggggatttaccacaccagacaaaaaacatcagaaagaacctccattcctttggatgggttatgaactccatcctgataaatggacagtacagcctatagtgctgccagaaaaggacagctggactgtcaatgacatacagaaattagtgggaaaattgaattgggcaagtcagatttatgcagggattaaagtaaggcaattatgtaaacttcttaggggaaccaaagcactaacagaagtagtaccactaacagaagaagcagagctagaactggcagaaaacagggagattctaaaagaaccggtacatggagtgtattatgacccatcaaaagacttaatagcagaaatacagaagcaggggcaaggccaatggacatatcaaatttatcaagagccatttaaaaatctgaaaacaggaaagtatgcaagaatgaagggtgcccacactaatgatgtgaaacaattaacagaggcagtacaaaaaatagccacagaaagcatagtaatatggggaaagactcctaaatttaaattacccatacaaaaggaaacatgggaagcatggtggacagagtattggcaagccacctggattcctgagtgggagtttgtcaatacccctcccttagtgaagttatggtaccagttagagaaagaacccataataggagcagaaactttctatgtagatggggcagccaatagggaaactaaattaggaaaagcaggatatgtaactgacagaggaagacaaaaagttgtccccctaacggacacaacaaatcagaagactgagttacaagcaattcatctagctttgcaggattcgggattagaagtaaacatagtgacagactcacaatatgcattgggaatcattcaagcacaaccagataagagtgaatcagagttagtcagtcaaataatagagcagttaataaaaaaggaaaaagtctacctggcatgggtaccagcacacaaaggaattggaggaaatgaacaagtagataaattggtcagtgctggaatcaggaaagtactatttttagatggaatagataaggcccaagaagaacatgagaaatatcacagtaattggagagcaatggctagtgattttaacctaccacctgtagtagcaaaagaaatagtagccagctgtgataaatgtcagctaaaaggggaagccatgcatggacaagtagactgtagcccaggaatatggcagctagattgtacacatttagaaggaaaagttatcttggtagcagttcatgtagccagtggatatatagaagcagaagtaattccagcagagacagggcaagaaacagcatacttcctcttaaaattagcaggaagatggccagtaaaaacagtacatacagacaatggcagcaatttcaccagtactacagttaaggccgcctgttggtgggcggggatcaagcaggaatttggcattccctacaatccgcagtcacaaggagtaatagaatctatgaataaagaattaaagaaaattataggacaggtaagagatcaggctgaacatcttaaaacagcagtacaaatggcagtattcatccacaattttaaaagaaaaggggggattggggggtacagtgcaggggaaagaatagtagacataatagcaacagacatacaaactaaagaattacaaaaacaaattacaaaaattcaaaattttcgggtttattacagggacagcagagatccagtttggaaaggaccagcaaagctcctctggaaaggtgaaggggcagtagtaatacaagataatagtgacataaaagtagtgccaagaagaaaagcaaagatcatcagggattatggaaaacagatggcaggtgatgattgtgtggcaagtagacaggatgaggattaacacatggaattccggagcggccgcaggagctttgttccttgggttcttgggagcagcaggaagcactatgggcgcagcgtcaatgacgctgacggtacaggccagacaattattgtctggtatagtgcagcagcagaacaatttgctgagggctattgaggcgcaacagcatctgttgcaactcacagtctggggcatcaagcagctccaggcaagaatcctggctgtggaaagatacctaaaggatcaacagctcctggggatttggggttgctctggaaaactcatttgcaccactgctgtgccttggaatgctagttggagtaataaatctctggaacagatttggaatcacacgacctggatggagtgggacagagaaattaacaattacacaagcttccgcggaattcaccccaccagtgcaggctgcctatcagaaagtggtggctggtgtggctaatgccctggcccacaagtatcactaagctcgctttcttgctgtccaatttctattaaaggttcctttgttccctaagtccaactactaaactgggggatattatgaagggccttgagcatctggattctgcctaataaaaaacatttattttcattgcaatgatgtatttaaattatttctgaatattttactaaaaagggaatgtgggaggtcagtgcatttaaaacataaagaaatgaagagctagttcaaaccttgggaaaatacactatatcttaaactccatgaaagaaggtgaggctgcaaacagctaatgcacattggcaacagcccctgatgcctatgccttattcatccctcagaaaaggattcaagtagaggcttgatttggaggttaaagttttgctatgctgtattttacattacttattgttttagctgtcctcatgaatgtcttttcactacccatttgcttatcctgcatctctcagccttgactccactcagttctcttgcttagagataccacctttcccctgaagtgttccttccatgttttacggcgagatggtttctcctcgcctggccactcagccttagttgtctctgttgtcttatagaggtctacttgaagaaggaaaaacagggggcatggtttgactgtcctgtgagcccttcttccctgcctcccccactcacagtgacccggaatccctcgacatggcagtctagcactagtgcggccgcagatctgcttcctcgctcactgactcgctgcgctcggtcgttcggctgcggcgagcggtatcagctcactcaaaggcggtaatacggttatccacagaatcaggggataacgcaggaaagaacatgtgagcaaaaggccagcaaaaggccaggaaccgtaaaaagtcgaccattacttattgttttagctgtcctcatgaatgtcttttcactacccatttgcttatcctgcatctctcagccttgactccactcagttctcttgcttagagataccacctttcccctgaagtgttccttccatgttttacggcgagatggtttctcctcgcctggccactcagccttagttgtctctgttgtcttatagaggtctacttgaagaaggaaaaacagggggcatggtttgactgtcctgtgagcccttcttccctgcctcccccactcacagtgacccggaatccctcgacatggcagtctagcactagtgcggccgcagatctgcttcctcgctcactgactcgctgcgctcggtcgttcggctgcggcgagcggtatcagctcactcaaaggcggtaatacggttatccacagaatcaggggataacgcaggaaagaacatgtgagcaaaaggccagcaaaaggccaggaaccgtaaaaa

SEQ ID NO: 20 - DNA, 7336 bp, synthetic construct
  misc_feature 1..7336: note = AAV2/8
  source 1..7336: mol_type = other DNA
atgccggggttttacgagattgtgattaaggtccccagcgaccttgacgagcatctgcccggcatttctgacagctttgtgaactgggtggccgagaaggaatgggagttgccgccagattctgacatggatctgaatctgattgagcaggcacccctgaccgtggccgagaagctgcagcgcgactttctgacggaatggcgccgtgtgagtaaggccccggaggctcttttctttgtgcaatttgagaagggagagagctacttccacatgcacgtgctcgtggaaaccaccggggtgaaatccatggttttgggacgtttcctgagtcagattcgcgaaaaactgattcagagaatttaccgcgggatcgagccgactttgccaaactggttcgcggtcacaaagaccagaaatggcgccggaggcgggaacaaggtggtggatgagtgctacatccccaattacttgctccccaaaacccagcctgagctccagtgggcgtggactaatatggaacagtatttaagcgcctgtttgaatctcacggagcgtaaacggttggtggcgcagcatctgacgcacgtgtcgcagacgcaggagcagaacaaagagaatcagaatcccaattctgatgcgccggtgatcagatcaaaaacttcagccaggtacatggagctggtcgggtggctcgtggacaaggggattacctcggagaagcagtggatccaggaggaccaggcctcatacatctccttcaatgcggcctccaactcgcggtcccaaatcaaggctgccttggacaatgcgggaaagattatgagcctgactaaaaccgcccccgactacctggtgggccagcagcccgtggaggacatttccagcaatcggatttataaaattttggaactaaacgggtacgatccccaatatgcggcttccgtctttctgggatgggccacgaaaaagttcggcaagaggaacaccatctggctgtttgggcctgcaactaccgggaagaccaacatcgcggaggccatagcccacactgtgcccttctacgggtgcgtaaactggaccaatgagaactttcccttcaacgactgtgtcgacaagatggtgatctggtgggaggaggggaagatgaccgccaaggtcgtggagtcggccaaagccattctcggaggaagcaaggtgcgcgtggaccagaaatgcaagtcctcggcccagatagacccgactcccgtgatcgtcacctccaacaccaacatgtgcgccgtgattgacgggaactcaacgaccttcgaacaccagcagccgttgcaagaccggatgttcaaatttgaactcacccgccgtctggatcatgactttgggaaggtcaccaagcaggaagtcaaagactttttccggtgggcaaaggatcacgtggttgaggtggagcatgaattctacgtcaaaaagggtggagccaagaaaagacccgcccccagtgacgcagatataagtgagcccaaacgggtgcgcgagtcagttgcgcagccatcgacgtcagacgcggaagcttcgatcaactacgcagacaggtaccaaaacaaatgttctcgtcacgtgggcatgaatctgatgctgtttccctgcagacaatgcgagagaatgaatcagaattcaaatatctgcttcactcacggacagaaagactgtttagagtgctttcccgtgtcagaatctcaacccgtttctgtcgtcaaaaaggcgtatcagaaactgtgctacattcatcatatcatgggaaaggtgccagacgcttgcactgcctgcgatctggtcaatgtggatttggatgactgcatctttgaacaataaatgatttaaatcaggtatggctgccgatggttatcttccagattggctcgaggacaacctctctgagggcattcgcgagtggtgggcgctgaaacctggagccccgaagcccaaagccaaccagcaaaagcaggacgacggccggggtctggtgcttcctggctacaagtacctcggacccttcaacggactcgacaagggggagcccgtcaacgcggcggacgcagcggccctcgagcacgacaaggcctacgaccagcagctgcaggcgggtgacaatccgtacctgcggtataaccacgccgacgccgagtttcaggagcgtctgcaagaagatacgtcttttgggggcaacctcgggcgagcagtcttccaggccaagaagcgggttctcgaacctctcggtctggttgaggaaggcgctaagacggctcctggaaagaagagaccggtagagccatcaccccagcgttctccagactcctctacgggcatcggcaagaaaggccaacagcccgccagaaaaagactcaattttggtcagactggcgactcagagtcagttccagaccctcaacctctcggagaacctccagcagcgccctctggtgtgggacctaatacaatggctgcaggcggtggcgcaccaatggcagacaataacgaaggcgccgacggagtgggtagttcctcgggaaattggcattgcgattccacatggctgggcgacagagtcatcaccaccagcacccgaacctgggccctgcccacctacaacaaccacctctacaagcaaatctccaacgggacatcgggaggagccaccaacgacaacacctacttcggctacagcaccccctgggggtattttgactttaacagattccactgccacttttcaccacgtgactggcagcgactcatcaacaacaactggggattccggcccaagagactcagcttcaagctcttcaacatccaggtcaaggaggtcacgcagaatgaaggcaccaagaccatcgccaataacctcaccagcaccatccaggtgtttacggactcggagtaccagctgccgtacgttctcggctctgcccaccagggctgcctgcctccgttcccggcggacgtgttcatgattccccagtacggctacctaacactcaacaacggtagtcaggccgtgggacgctcctccttctactgcctggaatactttccttcgcagatgctgagaaccggcaacaacttccagtttacttacaccttcgaggacgtgcctttccacagcagctacgcccacagccagagcttggaccggctgatgaatcctctgattgaccagtacctgtactacttgtctcggactcaaacaacaggaggcacggcaaatacgcagactctgggcttcagccaaggtgggcctaatacaatggccaatcaggcaaagaactggctgccaggaccctgttaccgccaacaacgcgtctcaacgacaaccgggcaaaacaacaatagcaactttgcctggactgctgggaccaaataccatctgaatggaagaaattcattggctaatcctggcatcgctatggcaacacacaaagacgacgaggagcgtttttttcccagtaacgggatcctgatttttggcaaacaaaatgctgccagagacaatgcggattacagcgatgtcatgctcaccagcgaggaagaaatcaaaaccactaaccctgtggctacagaggaatacggtatcgtggcagataacttgcagcagcaaaacacggctcctcaaattggaactgtcaacagccagggggccttacccggtatggtctggcagaaccgggacgtgtacctgcagggtcccatctgggccaagattcctcacacggacggcaacttccacccgtctccgctgatgggcggctttggcctgaaacatcctccgcctcagatcctgatcaagaacacgcctgtacctgcggatcctccgaccaccttcaaccagtcaaagctgaactctttcatcacgcaatacagcaccggacaggtcagcgtggaaattgaatgggagctgcagaaggaaaacagcaagcgctggaaccccgagatccagtacacctccaactactacaaatctacaagtgtggactttgctgttaatacagaaggcgtgtactctgaaccccgccccattggcacccgttacctcacccgtaatctgtaattgcctgttaatcaataaaccggttgattcgtttcagttgaactttggtctctgcgaagggcgaattcgtttaaacctgcaggactagaggtcctgtattagaggtcacgtgagtgttttgcgacattttgcgacaccatgtggtcacgctgggtatttaagcccgagtgagcacgcagggtctccattttgaagcgggaggtttgaacgcgcagccgccaagccgaattctgcagatatccatcacactggcggccgctcgactagagcggccgccaccgcggtggagctccagcttttgttccctttagtgagggttaattgcgcgcttggcgtaatcatggtcatagctgtttcctgtgtgaaattgttatccgctcacaattccacacaacatacgagccggaagcataaagtgtaaagcctggggtgcctaatgagtgagctaactcacattaattgcgttgcgctcactgcccgctttccagtcgggaaacctgtcgtgccagctgcattaatgaatcggccaacgcgcggggagaggcggtttgcgtattgggcgctcttccgcttcctcgctcactgactcgctgcgctcggtcgttcggctgcggcgagcggtatcagctcactcaaaggcggtaatacggttatccacagaatcaggggataacgcaggaaagaacatgtgagcaaaaggccagcaaaaggccaggaaccgtaaaaaggccgcgttgctggcgtttttccataggctccgcccccctgacgagcatcacaaaaatcgacgctcaagtcagaggtggcgaaacccgacaggactataaagataccaggcgtttccccctggaagctccctcgtgcgctctcctgttccgaccctgccgcttaccggatacctgtccgcctttctcccttcgggaagcgtggcgctttctcatagctcacgctgtaggtatctcagttcggtgtaggtcgttcgctccaagctgggctgtgtgcacgaaccccccgttcagcccgaccgctgcgccttatccggtaactatcgtcttgagtccaacccggtaagacacgacttatcgccactggcagcagccactggtaacaggattagcagagcgaggtatgtaggcggtgctacagagttcttgaagtggtggcctaactacggctacactagaagaacagtatttggtatctgcgctctgctgaagccagttaccttcggaaaaagagttggtagctcttgatccggcaaacaaaccaccgctggtagcggtggtttttttgtttgcaagcagcagattacgcgcagaaaaaaaggatctcaagaagatcctttgatcttttctacggggtctgacgctcagtggaacgaaaactcacgttaagggattttggtcatgagattatcaaaaaggatcttcacctagatccttttaaattaaaaatgaagttttaaatcaatctaaagtatatatgagtaaacttggtctgacagttaccaatgcttaatcagtgaggcacctatctcagcgatctgtctatttcgttcatccatagttgcctgactccccgtcgtgtagataactacgatacgggagggcttaccatctggccccagtgctgcaatgataccgcgagacccacgctcaccggctccagatttatcagcaataaaccagccagccggaagggccgagcgcagaagtggtcctgcaactttatccgcctccatccagtctattaattgttgccgggaagctagagtaagtagttcgccagttaatagtttgcgcaacgttgttgccattgctacaggcatcgtggtgtcacgctcgtcgtttggtatggcttcattcagctccggttcccaacgatcaaggcgagttacatgatcccccatgttgtgcaaaaaagcggttagctccttcggtcctccgatcgttgtcagaagtaagttggccgcagtgttatcactcatggttatggcagcactgcataattctcttactgtcatgccatccgtaagatgcttttctgtgactggtgagtactcaaccaagtcattctgagaatagtgtatgcggcgaccgagttgctcttgcccggcgtcaatacgggataataccgcgccacatagcagaactttaaaagtgctcatcattggaaaacgttcttcggggcgaaaactctcaaggatcttaccgctgttgagatccagttcgatgtaacccactcgtgcacccaactgatcttcagcatcttttactttcaccagcgtttctgggtgagcaaaaacaggaaggcaaaatgccgcaaaaaagggaataagggcgacacggaaatgttgaatactcatactcttcctttttcaatattattgaagcatttatcagggttattgtctcatgagcggatacatatttgaatgtatttagaaaaataaacaaataggggttccgcgcacatttccccgaaaagtgccacctaaattgtaagcgttaatattttgttaaaattcgcgttaaatttttgttaaatcagctcattttttaaccaataggccgaaatcggcaaaatcccttataaatcaaaagaatagaccgagatagggttgagtgttgttccagtttggaacaagagtccactattaaagaacgtggactccaacgtcaaagggcgaaaaaccgtctatcagggcgatggcccactacgtgaaccatcaccctaatcaagttttttggggtcgaggtgccgtaaagcactaaatcggaaccctaaagggagcccccgatttagagcttgacggggaaagccggcgaacgtggcgagaaaggaagggaagaaagcgaaaggagcgggcgctagggcgctggcaagtgtagcggtcacgctgcgcgtaaccaccacacccgccgcgcttaatgcgccgctacagggcgcgtcccattcgccattcaggctgcgcaactgttgggaagggcgatcggtgcgggcctcttcgctattacgccagctggcgaaagggggatgtgctgcaaggcgattaagttgggtaacgccagggttttcccagtcacgacgttgtaaaacgacggccagtgagcgcgcgtaatacgactcactatagggcgaattgggtaccgggccccccctcgatcgaggtcgacggtatcgggggagctcgcagggtctccattttgaagcgggaggtttgaacgcgcagccgcc

SEQ ID NO: 21 - DNA, 11635 bp, synthetic construct
  misc_feature 1..11635: note = pHelper
  source 1..11635: mol_type = other DNA
ggtacccaactccatgcttaacagtccccaggtacagcccaccctgcgtcgcaaccaggaacagctctacagcttcctggagcgccactcgccctacttccgcagccacagtgcgcagattaggagcgccacttctttttgtcacttgaaaaacatgtaaaaataatgtactaggagacactttcaataaaggcaaatgtttttatttgtacactctcgggtgattatttaccccccacccttgccgtctgcgccgtttaaaaatcaaaggggttctgccgcgcatcgctatgcgccactggcagggacacgttgcgatactggtgtttagtgctccacttaaactcaggcacaaccatccgcggcagctcggtgaagttttcactccacaggctgcgcaccatcaccaacgcgtttagcaggtcgggcgccgatatcttgaagtcgcagttggggcctccgccctgcgcgcgcgagttgcgatacacagggttgcagcactggaacactatcagcgccgggtggtgcacgctggccagcacgctcttgtcggagatcagatccgcgtccaggtcctccgcgttgctcagggcgaacggagtcaactttggtagctgccttcccaaaaagggtgcatgcccaggctttgagttgcactcgcaccgtagtggcatcagaaggtgaccgtgcccggtctgggcgttaggatacagcgcctgcatgaaagccttgatctgcttaaaagccacctgagcctttgcgccttcagagaagaacatgccgcaagacttgccggaaaactgattggccggacaggccgcgtcatgcacgcagcaccttgcgtcggtgttggagatctgcaccacatttcggccccaccggttcttcacgatcttggccttgctagactgctccttcagcgcgcgctgcccgttttcgctcgtcacatccatttcaatcacgtgctccttatttatcataatgctcccgtgtagacacttaagctcgccttcgatctcagcgcagcggtgcagccacaacgcgcagcccgtgggctcgtggtgcttgtaggttacctctgcaaacgactgcaggtacgcctgcaggaatcgccccatcatcgtcacaaaggtcttgttgctggtgaaggtcagctgcaacccgcggtgctcctcgtttagccaggtcttgcatacggccgccagagcttccacttggtcaggcagtagcttgaagtttgcctttagatcgttatccacgtggtacttgtccatcaacgcgcgcgcagcctccatgcccttctcccacgcagacacgatcggcaggctcagcgggtttatcaccgtgctttcactttccgcttcactggactcttccttttcctcttgcgtccgcataccccgcgccactgggtcgtcttcattcagccgccgcaccgtgcgcttacctcccttgccgtgcttgattagcaccggtgggttgctgaaacccaccatttgtagcgccacatcttctctttcttcctcgctgtccacgatcacctctggggatggcgggcgctcgggcttgggagaggggcgcttctttttctttttggacgcaatggccaaatccgccgtcgaggtcgatggccgcgggctgggtgtgcgcggcaccagcgcatcttgtgacgagtcttcttcgtcctcggactcgagacgccgcctcagccgcttttttgggggcgcgcggggaggcggcggcgacggcgacggggacgacacgtcctccatggttggtggacgtcgcgccgcaccgcgtccgcgctcgggggtggtttcgcgctgctcctcttcccgactggccatttccttctcctataggcagaaaaagatcatggagtcagtcgagaaggaggacagcctaaccgccccctttgagttcgccaccaccgcctccaccgatgccgccaacgcgcctaccaccttccccgtcgaggcacccccgcttgaggaggaggaagtgattatcgagcaggacccaggttttgtaagcgaagacgacgaggatcgctcagtaccaacagaggataaaaagcaagaccaggacgacgcagaggcaaacgaggaacaagtcgggcggggggaccaaaggcatggcgactacctagatgtgggagacgacgtgctgttgaagcatctgcagcgccagtgcgccattatctgcgacgcgttgcaagagcgcagcgatgtgcccctcgccatagcggatgtcagccttgcctacgaacgccacctgttctcaccgcgcgtaccccccaaacgccaagaaaacggcacatgcgagcccaacccgcgcctcaacttctaccccgtatttgccgtgccagaggtgcttgccacctatcacatctttttccaaaactgcaagatacccctatcctgccgtgccaaccgcagccgagcggacaagcagctggccttgcggcagggcgctgtcatacctgatatcgcctcgctcgacgaagtgccaaaaatctttgagggtcttggacgcgacgagaaacgcgcggcaaacgctctgcaacaagaaaacagcgaaaatgaaagtcactgtggagtgctggtggaacttgagggtgacaacgcgcgcctagccgtgctgaaacgcagcatcgaggtcacccactttgcctacccggcacttaacctaccccccaaggttatgagcacagtcatgagcgagctgatcgtgcgccgtgcacgacccctggagagggatgcaaacttgcaagaacaaaccgaggagggcctacccgcagttggcgatgagcagctggcgcgctggcttgagacgcgcgagcctgccgacttggaggagcgacgcaagctaatgatggccgcagtgcttgttaccgtggagcttgagtgcatgcagcggttctttgctgacccggagatgcagcgcaagctagaggaaacgttgcactacacctttcgccagggctacgtgcgccaggcctgcaaaatttccaacgtggagctctgcaacctggtctcctaccttggaattttgcacgaaaaccgcctcgggcaaaacgtgcttcattccacgctcaagggcgaggcgcgccgcgactacgtccgcgactgcgtttacttatttctgtgctacacctggcaaacggccatgggcgtgtggcagcaatgcctggaggagcgcaacctaaaggagctgcagaagctgctaaagcaaaacttgaaggacctatggacggccttcaacgagcgctccgtggccgcgcacctggcggacattatcttccccgaacgcctgcttaaaaccctgcaacagggtctgccagacttcaccagtcaaagcatgttgcaaaactttaggaactttatcctagagcgttcaggaattctgcccgccacctgctgtgcgcttcctagcgactttgtgcccattaagtaccgtgaatgccctccgccgctttggggtcactgctaccttctgcagctagccaactaccttgcctaccactccgacatcatggaagacgtgagcggtgacggcctactggagtgtcactgtcgctgcaacctatgcaccccgcaccgctccctggtctgcaattcgcaactgcttagcgaaagtcaaattatcggtacctttgagctgcagggtccctcgcctgacgaaaagtccgcggctccggggttgaaactcactccggggctgtggacgtcggcttaccttcgcaaatttgtacctgaggactaccacgcccacgagattaggttctacgaagaccaatcccgcccgccaaatgcggagcttaccgcctgcgtcattacccagggccacatccttggccaattgcaagccatcaacaaagcccgccaagagtttctgctacgaaagggacggggggtttacctggacccccagtccggcgaggagctcaacccaatccccccgccgccgcagccctatcagcagccgcgggcccttgcttcccaggatggcacccaaaaagaagctgcagctgccgccgccgccacccacggacgaggaggaatactgggacagtcaggcagaggaggttttggacgaggaggaggagatgatggaagactgggacagcctagacgaagcttccgaggccgaagaggtgtcagacgaaacaccgtcaccctcggtcgcattcccctcgccggcgccccagaaattggcaaccgttcccagcatcgctacaacctccgctcctcaggcgccgccggcactgcctgttcgccgacccaaccgtagatgggacaccactggaaccagggccggtaagtctaagcagccgccgccgttagcccaagagcaacaacagcgccaaggctaccgctcgtggcgcgggcacaagaacgccatagttgcttgcttgcaagactgtgggggcaacatctccttcgcccgccgctttcttctctaccatcacggcgtggccttcccccgtaacatcctgcattactaccgtcatctctacagcccctactgcaccggcggcagcggcagcggcagcaacagcagcggtcacacagaagcaaaggcgaccggatagcaagactctgacaaagcccaagaaatccacagcggcggcagcagcaggaggaggagcgctgcgtctggcgcccaacgaacccgtatcgacccgcgagcttagaaataggatttttcccactctgtatgctatatttcaacaaagcaggggccaagaacaagagctgaaaataaaaaacaggtctctgcgctccctcacccgcagctgcctgtatcacaaaagcgaagatcagcttcggcgcacgctggaagacgcggaggctctcttcagcaaatactgcgcgctgactcttaaggactagtttcgcgccctttctcaaatttaagcgcgaaaactacgtcatctccagcggccacacccggcgccagcacctgtcgtcagcgccattatgagcaaggaaattcccacgccctacatgtggagttaccagccacaaatgggacttgcggctggagctgcccaagactactcaacccgaataaactacatgagcgcgggaccccacatgatatcccgggtcaacggaatccgcgcccaccgaaaccgaattctcctcgaacaggcggctattaccaccacacctcgtaataaccttaatccccgtagttggcccgctgccctggtgtaccaggaaagtcccgctcccaccactgtggtacttcccagagacgcccaggccgaagttcagatgactaactcaggggcgcagcttgcgggcggctttcgtcacagggtgcggtcgcccgggcgttttagggcggagtaacttgcatgtattgggaattgtagtttttttaaaatgggaagtgacgtatcgtgggaaaacggaagtgaagatttgaggaagttgtgggttttttggctttcgtttctgggcgtaggttcgcgtgcggttttctgggtgttttttgtggactttaaccgttacgtcattttttagtcctatatatactcgctctgtacttggccctttttacactgtgactgattgagctggtgccgtgtcgagtggtgttttttaataggtttttttactggtaaggctgactgttatggctgccgctgtggaagcgctgtatgttgttctggagcgggagggtgctattttgcctaggcaggagggtttttcaggtgtttatgtgtttttctctcctattaattttgttatacctcctatgggggctgtaatgttgtctctacgcctgcgggtatgtattcccccgggctatttcggtcgctttttagcactgaccgatgttaaccaacctgatgtgtttaccgagtcttacattatgactccggacatgaccgaggaactgtcggtggtgctttttaatcacggtgaccagtttttttacggtcacgccggcatggccgtagtccgtcttatgcttataagggttgtttttcctgttgtaagacaggcttctaatgtttaaatgtttttttttttgttattttattttgtgtttaatgcaggaacccgcagacatgtttgagagaaaaatggtgtctttttctgtggtggttccggaacttacctgcctttatctgcatgagcatgactacgatgtgcttgcttttttgcgcgaggctttgcctgattttttgagcagcaccttgcattttatatcgccgcccatgcaacaagcttacataggggctacgctggttagcatagctccgagtatgcgtgtcataatcagtgtgggttcttttgtcatggttcctggcggggaagtggccgcgctggtccgtgcagacctgcacgattatgttcagctggccctgcgaagggacctacgggatcgcggtatttttgttaatgttccgcttttgaatcttatacaggtctgtgaggaacctgaatttttgcaatcatgattcgctgcttgaggctgaaggtggagggcgctctggagcagatttttacaatggccggacttaatattcgggatttgcttagagacatattgataaggtggcgagatgaaaattatttgggcatggttgaaggtgctggaatgtttatagaggagattcaccctgaagggtttagcctttacgtccacttggacgtgagggcagtttgccttttggaagccattgtgcaacatcttacaaatgccattatctgttctttggctgtagagtttgaccacgccaccggaggggagcgcgttcacttaatagatcttcattttgaggttttggataatcttttggaataaaaaaaaaaaaacatggttcttccagctcttcccgctcctcccgtgtgtgactcgcagaacgaatgtgtaggttggctgggtgtggcttattctgcggtggtggatgttatcagggcagcggcgcatgaaggagtttacatagaacccgaagccagggggcgcctggatgctttgagagagtggatatactacaactactacacagagcgagctaagcgacgagaccggagacgcagatctgtttgtcacgcccgcacctggttttgcttcaggaaatatgactacgtccggcgttccatttggcatgacactacgaccaacacgatctcggttgtctcggcgcactccgtacagtagggatcgcctacctccttttgagacagagacccgcgctaccatactggaggatcatccgctgctgcccgaatgtaacactttgacaatgcacaacgtgagttacgtgcgaggtcttccctgcagtgtgggatttacgctgattcaggaatgggttgttccctgggatatggttctgacgcgggaggagcttgtaatcctgaggaagtgtatgcacgtgtgcctgtgttgtgccaacattgatatcatgacgagcatgatgatccatggttacgagtcctgggctctccactgtcattgttccagtcccggttccctgcagtgcatagccggcgggcaggttttggccagctggtttaggatggtggtggatggcgccatgtttaatcagaggtttatatggtaccgggaggtggtgaattacaacatgccaaaagaggtaatgtttatgtccagcgtgtttatgaggggtcgccacttaatctacctgcgcttgtggtatgatggccacgtgggttctgtggtccccgccatgagctttggatacagcgccttgcactgtgggattttgaacaatattgtggtgctgtgctgcagttactgtgctgatttaagtgagatcagggtgcgctgctgtgcccggaggacaaggcgtctcatgctgcgggcggtgcgaatcatcgctgaggagaccactgccatgttgtattcctgcaggacggagcggcggcggcagcagtttattcgcgcgctgctgcagcaccaccgccctatcctgatgcacgattatgactctacccccatgtaggcgtggacttccccttcgccgcccgttgagcaaccgcaagttggacagcagcctgtggctcagcagctggacagcgacatgaacttaagcgagctgcccggggagtttattaatatcactgatgagcgtttggctcgacaggaaaccgtgtggaatataacacctaagaatatgtctgttacccatgatatgatgctttttaaggccagccggggagaaaggactgtgtactctgtgtgttgggagggaggtggcaggttgaatactagggttctgtgagtttgattaaggtacggtgatcaatataagctatgtggtggtggggctatactactgaatgaaaaatgacttgaaattttctgcaattgaaaaataaacacgttgaaacataacatgcaacaggttcacgattctttattcctgggcaatgtaggagaaggtgtaagagttggtagcaaaagtttcagtggtgtattttccactttcccaggaccatgtaaaagacatagagtaagtgcttacctcgctagtttctgtggattcactagaatcgatgtaggatgttgcccctcctgacgcggtaggagaaggggagggtgccctgcatgtctgccgctgctcttgctcttgccgctgctgaggaggggggcgcatctgccgcagcaccggatgcatctgggaaaagcaaaaaaggggctcgtccctgtttccggaggaatttgcaagcggggtcttgcatgacggggaggcaaacccccgttcgccgcagtccggccggcccgagactcgaaccgggggtcctgcgactcaacccttggaaaataaccctccggctacagggagcgagccacttaatgctttcgctttccagcctaaccgcttacgccgcgcgcggccagtggccaaaaaagctagcgcagcagccgccgcgcctggaaggaagccaaaaggagcgctcccccgttgtctgacgtcgcacacctgggttcgacacgcgggcggtaaccgcatggatcacggcggacggccggatccggggttcgaaccccggtcgtccgccatgatacccttgcgaatttatccaccagaccacggaagagtgcccgcttacaggctctccttttgcacggtctagagcgtcaacgactgcgcacgcctcaccggccagagcgtcccgaccatggagcactttttgccgctgcgcaacatctggaaccgcgtccgcgactttccgcgcgcctccaccaccgccgccggcatcacctggatgtccaggtacatctacggattacgtcgacgtttaaaccatatgatcagctcactcaaaggcggtaatacggttatccacagaatcaggggataacgcaggaaagaacatgtgagcaaaaggccagcaaaaggccaggaaccgtaaaaaggccgcgttgctggcgtttttccataggctccgcccccctgacgagcatcacaaaaatcgacgctcaagtcagaggtggcgaaacccgacaggactataaagataccaggcgtttccccctggaagctccctcgtgcgctctcctgttccgaccctgccgcttaccggatacctgtccgcctttctcccttcgggaagcgtggcgctttctcatagctcacgctgtaggtatctcagttcggtgtaggtcgttcgctccaagctgggctgtgtgcacgaaccccccgttcagcccgaccgctgcgccttatccggtaactatcgtcttgagtccaacccggtaagacacgacttatcgccactggcagcagccactggtaacaggattagcagagcgaggtatgtaggcggtgctacagagttcttgaagtggtggcctaactacggctacactagaagaacagtatttggtatctgcgctctgctgaagccagttaccttcggaaaaagagttggtagctcttgatccggcaaacaaaccaccgctggtagcggtggtttttttgtttgcaagcagcagattacgcgcagaaaaaaaggatctcaagaagatcctttgatcttttctacggggtctgacgctcagtggaacgaaaactcacgttaagggattttggtcatgagattatcaaaaaggatcttcacctagatccttttaaattaaaaatgaagttttaaatcaatctaaagtatatatgagtaaacttggtctgacagttaccaatgcttaatcagtgaggcacctatctcagcgatctgtctatttcgttcatccatagttgcctgactccccgtcgtgtagataactacgatacgggagggcttaccatctggccccagtgctgcaatgataccgcgagacccacgctcaccggctccagatttatcagcaataaaccagccagccggaagggccgagcgcagaagtggtcctgcaactttatccgcctccatccagtctattaattgttgccgggaagctagagtaagtagttcgccagttaatagtttgcgcaacgttgttgccattgctacaggcatcgtggtgtcacgctcgtcgtttggtatggcttcattcagctccggttcccaacgatcaaggcgagttacatgatcccccatgttgtgcaaaaaagcggttagctccttcggtcctccgatcgttgtcagaagtaagttggccgcagtgttatcactcatggttatggcagcactgcataattctcttactgtcatgccatccgtaagatgcttttctgtgactggtgagtactcaaccaagtcattctgagaatagtgtatgcggcgaccgagttgctcttgcccggcgtcaatacgggataataccgcgccacatagcagaactttaaaagtgctcatcattggaaaacgttcttcggggcgaaaactctcaaggatcttaccgctgttgagatccagttcgatgtaacccactcgtgcacccaactgatcttcagcatcttttactttcaccagcgtttctgggtgagcaaaaacaggaaggcaaaatgccgcaaaaaagggaataagggcgacacggaaatgttgaatactcatactcttcctttttcaatattattgaagcatttatcagggttattgtctcatgagcggatacatatttgaatgtatttagaaaaataaacaaataggggttccgcgcacatttccccgaaaagtgccacctaaattgtaagcgttaatattttgttaaaattcgcgttaaatttttgttaaatcagctcattttttaaccaataggccgaaatcggcaaaatcccttataaatcaaaagaatagaccgagatagggttgagtgttgttccagtttggaacaagagtccactattaaagaacgtggactccaacgtcaaagggcgaaaaaccgtctatcagggcgatggcccactacgtgaaccatcaccctaatcaagttttttggggtcgaggtgccgtaaagcactaaatcggaaccctaaagggagcccccgatttagagcttgacggggaaagccggcgaacgtggcgagaaaggaagggaagaaagcgaaaggagcgggcgctagggcgctggcaagtgtagcggtcacgctgcgcgtaaccaccacacccgccgcgcttaatgcgccgctacagggcgcgatggatcc

SEQ ID NO: 22 - DNA, 814 bp, synthetic construct
  source 1..814: mol_type = other DNA; note = CBH promoter
cgttacataacttacggtaaatggcccgcctggctgaccgcccaacgacccccgcccattgacgtcaataatgacgtatgttcccatagtaacgccaatagggactttccattgacgtcaatgggtggagtatttacggtaaactgcccacttggcagtacatcaagtgtatcatatgccaagtacgccccctattgacgtcaatgacggtaaatggcccgcctggcattatgcccagtacatgaccttatgggactttcctacttggcagtacatctacgtattagtcatcgctattaccatggtcgaggtgagccccacgttctgcttcactctccccatctcccccccctccccacccccaattttgtatttatttattttttaattattttgtgcagcgatgggggcggggggggggggggggcgcgcgccaggcggggcggggcggggcgaggggcggggcggggcgaggcggagaggtgcggcggcagccaatcagagcggcgcgctccgaaagtttccttttatggcgaggcggcggcggcggcggccctataaaaagcgaagcgcgcggcgggcgggagtcgctgcgacgctgccttcgccccgtgccccgctccgccgccgcctcgcgccgcccgccccggctctgactgaccgcgttactcccacaggtgagcgggcgggacggcccttctcctccgggctgtaattagctgagcaagaggtaagggtttaagggatggttggttggtggggtattaatgtttaattacctggagcacctgcctgaaatcactttttttcaggt